European Patent Specification EP 4 274 893 B1, published January 1, 2025. Title: Method for producing genetically modified cells. Applicant: Horizon Discovery Limited Dharmacon, Inc. The sequence listing filed with the application follows.

SEQUENCE LISTING (73 sequences)

SEQ ID NO: 1 - RNA, 42 nt, Artificial Sequence
  Type II crRNA seq
  misc_feature (1)..(20): n is a, c, g, or u
nnnnnnnnnnnnnnnnnnnnguuuuagagcuaugcuguuuug

SEQ ID NO: 2 - RNA, 99 nt, Artificial Sequence
  Type II tracrRNA seq
aacagcauagcaaguuaaaauaaggcuaguccguuaucaacuugaaaaaguggcaccgagucggugcgcgcacaugaggaucacccaugugcuuuuuuu

SEQ ID NO: 3 - DNA, 44 bp, Artificial Sequence
  AsCas12a crRNA Targets PPIB seq
uaauuucuacucuuguagauacctacgaattggagatgaagatg

SEQ ID NO: 4 - DNA, 158 bp, Artificial Sequence
  AaCas12b sgRNA - Targets PPIB seq
ggtctaaaggacagaatttttcaacgggtgtgccaatggccactttccaggtggcaaagcccgttgaacttctcaaaaagaacgctcgctcagtgttctgacgtcggatcactgagcgagcgatctgagaagtggcacacctacgaattggagatgaa

SEQ ID NO: 5 - RNA, 70 nt, Artificial Sequence
  Cas12d15 scoutRNA seq
cuuaguuaaggauguuccagguucuuucgggagccuuggccuucucccuuaaccuaugccacuaaugauu

SEQ ID NO: 6 - DNA, 45 bp, Artificial Sequence
  Cas12d15 crRNA - Targets PPIB seq
acccguaaagcagagcgaugaaggcacctacgaattggagatgaa

SEQ ID NO: 7 - RNA, 66 nt, Artificial Sequence
  Telomerase Ku binding motif / Ku heterodimer - Ku binding hairpin seq
uucuugucguacuuauagaucgcuacguuauuucaauuuugaaaaucugaguccugggagugcgga

SEQ ID NO: 8 - protein, 1094 aa, Artificial Sequence
  Telomerase Ku binding motif / Ku heterodimer - Ku heterodimer seq
MSGWESYYKTEGDEEAEEEQEENLEASGDYKYSGRDSLIFLVDASKAMFESQSEDELTPFDMSIQCIQSVYISKIISSDRDLLAVVFYGTEKDKNSVNFKNIYVLQELDNPGAKRILELDQFKGQQGQKRFQDMMGHGSDYSLSEVLWVCANLFSDVQFKMSHKRIMLFTNEDNPHGNDSAKASRARTKAGDLRDTGIFLDLMHLKKPGGFDISLFYRDIISIAEDEDLRVHFEESSKLEDLLRKVRAKETRKRALSRLKLKLNKDIVISVGIYNLVQKALKPPPIKLYRETNEPVKTKTRTFNTSTGGLLLPSDTKRSQIYGSRQIILEKEETEELKRFDDPGLMLMGFKPLVLLKKHHYLRPSLFVYPEESLVIGSSTLFSALLIKCLEKEVAALCRYTPRRNIPPYFVALVPQEEELDDQKIQVTPPGFQLVFLPFADDKRKMPFTEKIMATPEQVGKMKAIVEKLRFTYRSDSFENPVLQQHFRNLEALALDLMEPEQAVDLTLPKVEAMNKRLGSLVDEFKELVYPPDYNPEGKVTKRKHDNEGSGSKRPKVEYSEEELKTHISKGTLGKFTVPMLKEACRAYGLKSGLKKQELLEALTKHFQDMVRSGNKAAVVLCMDVGFTMSNSIPGIESPFEQAKKVITMFVQRQVFAENKDEIALVLFGTDGTDNPLSGGDQYQNITVHRHLMLPDFDLLEDIESKIQPGSQQADFLDALIVSMDVIQHETIGKKFEKRHIEIFTDLSSRFSKSQLDIIIHSLKKCDISERHSIHWPCRLTIGSNLSIRIAAYKSILQERVKKTWTVVDAKTLKKEDIQKETVYCLNDDDETEVLKEDIIQGFRYGSDIVPFSKVDEEQMKYKSEGKCFSVLGFCKSSQVQRRFFMGNQVLKVFAARDDEAAAVALSSLIHALDDLDMVAIVRYAYDKRANPQVGVAFPHIKHNYECLVYVQLPFMEDLRQYMFSSLKNSKKYAPTEAQLNAVDALIDSMSLAKKDEKTDTLEDLFPTTKIPNPRFQRLFQCLLHRALHPREPLPPIQQHIWNMLNPPAEVTTKSQIPLSKIKTLFPLIEAKKKDQVTAQEIFQDNHEDGPTAK

SEQ ID NO: 9 - RNA, 10 nt, Artificial Sequence
  Telomerase Sm7 binding motif / Sm7 homoheptamer - Sm consensus site seq
aauuuuugga

SEQ ID NO: 10 - protein, 83 aa, Artificial Sequence
  Telomerase Sm7 binding motif / Sm7 homoheptamer - Monomeric Sm - like protein (archaea)
GSVIDVSSQRVNVQRPLDALGNSLNSPVIIKLKGDREFRGVLKSFDLHMNLVLNDAEELEDGEVTRRLGTVLIRGDNIVYISP

SEQ ID NO: 11 - RNA, 25 nt, Artificial Sequence
  MS2 phage operator stem loop / MS2 coat protein - MS2 phage operator stem loop seq
gcgcacaugaggaucacccaugugc

SEQ ID NO: 12 - protein, 117 aa, Artificial Sequence
  MS2 phage operator stem loop / MS2 coat protein - MS2 coat protein
MASNFTQFVLVDNGGTGDVTVAPSNFANGIAEWISSNSRSQAYKVTCSVRQSSAQNRKYTIKVEVPKGAWRSYLNMELTIPIFATNSDCELIVKAMQGLLKDGNPIPSAIAANSGIY

SEQ ID NO: 13 - RNA, 25 nt, Artificial Sequence
  PP7 phage operator stem loop / PP7 coat protein - PP7 phage operator stem loop seq
auaaggaguuuauauggaaacccuu

SEQ ID NO: 14 - protein, 128 aa, Artificial Sequence
  PP7 phage operator stem loop / PP7 coat protein - PP7 coat protein (PCP) seq
MSKTIVLSVGEATRTLTEIQSTADRQIFEEKVGPLVGRLRLTASLRQNGAKTAYRVNLKLDQADVVDCSTSVCGELPKVRYTQVWSHDVTIVANSTEASRKSLYDLTKSLVATSQVEDLVVNLVPLGR

SEQ ID NO: 15 - RNA, 19 nt, Artificial Sequence
  SfMu Com stem loop / SfMu Com binding protein - SfMu Com stem loop seq
cugaaugccugcgagcauc

SEQ ID NO: 16 - protein, 62 aa, Artificial Sequence
  SfMu Com stem loop / SfMu Com binding protein - SfMu Com binding protein seq
MKSIRCKNCNKLLFKADSFDHIEIRCPRCKRHIIMLNACEHPTEKHCGKREKITHSDETVRY

SEQ ID NO: 17 - protein, 1368 aa, Artificial Sequence
  Humanised amino acid sequence Streptococcus pyogenes dCas9 seq
MDKKYSIGLAIGTNSVGWAVITDEYKVPSKKFKVLGNTDRHSIKKNLIGALLFDSGETAEATRLKRTARRRYTRRKNRICYLQEIFSNEMAKVDDSFFHRLEESFLVEEDKKHERHPIFGNIVDEVAYHEKYPTIYHLRKKLVDSTDKADLRLIYLALAHMIKFRGHFLIEGDLNPDNSDVDKLFIQLVQTYNQLFEENPINASGVDAKAILSARLSKSRRLENLIAQLPGEKKNGLFGNLIALSLGLTPNFKSNFDLAEDAKLQLSKDTYDDDLDNLLAQIGDQYADLFLAAKNLSDAILLSDILRVNTEITKAPLSASMIKRYDEHHQDLTLLKALVRQQLPEKYKEIFFDQSKNGYAGYIDGGASQEEFYKFIKPILEKMDGTEELLVKLNREDLLRKQRTFDNGSIPHQIHLGELHAILRRQEDFYPFLKDNREKIEKILTFRIPYYVGPLARGNSRFAWMTRKSEETITPWNFEEVVDKGASAQSFIERMTNFDKNLPNEKVLPKHSLLYEYFTVYNELTKVKYVTEGMRKPAFLSGEQKKAIVDLLFKTNRKVTVKQLKEDYFKKIECFDSVEISGVEDRFNASLGTYHDLLKIIKDKDFLDNEENEDILEDIVLTLTLFEDREMIEERLKTYAHLFDDKVMKQLKRRRYTGWGRLSRKLINGIRDKQSGKTILDFLKSDGFANRNFMQLIHDDSLTFKEDIQKAQVSGQGDSLHEHIANLAGSPAIKKGILQTVKVVDELVKVMGRHKPENIVIEMARENQTTQKGQKNSRERMKRIEEGIKELGSQILKEHPVENTQLQNEKLYLYYLQNGRDMYVDQELDINRLSDYDVDAIVPQSFLKDDSIDNKVLTRSDKNRGKSDNVPSEEVVKKMKNYWRQLLNAKLITQRKFDNLTKAERGGLSELDKAGFIKRQLVETRQITKHVAQILDSRMNTKYDENDKLIREVKVITLKSKLVSDFRKDFQFYKVREINNYHHAHDAYLNAVVGTALIKKYPKLESEFVYGDYKVYDVRKMIAKSEQEIGKATAKYFFYSNIMNFFKTEITLANGEIRKRPLIETNGETGEIVWDKGRDFATVRKVLSMPQVNIVKKTEVQTGGFSKESILPKRNSDKLIARKKDWDPKKYGGFDSPTVAYSVLVVAKVEKGKSKKLKSVKELLGITIMERSSFEKNPIDFLEAKGYKEVKKDLIIKLPKYSLFELENGRKRMLASAGELQKGNELALPSKYVNFLYLASHYEKLKGSPEDNEQKQLFVEQHKHYLDEIIEQISEFSKRVILADANLDKVLSAYNKHRDKPIREQAENIIHLFTLTNLGAPAAFKYFDTTIDRKRYTSTKEVLDATLIHQSITGLYETRIDLSQLGGD

SEQ ID NO: 18 - protein, 1367 aa, Artificial Sequence
  Cas9 D10A Amino Acid Sequence
DKKYSIGLAIGTNSVGWAVITDEYKVPSKKFKVLGNTDRHSIKKNLIGALLFDSGETAEATRLKRTARRRYTRRKNRICYLQEIFSNEMAKVDDSFFHRLEESFLVEEDKKHERHPIFGNIVDEVAYHEKYPTIYHLRKKLVDSTDKADLRLIYLALAHMIKFRGHFLIEGDLNPDNSDVDKLFIQLVQTYNQLFEENPINASGVDAKAILSARLSKSRRLENLIAQLPGEKKNGLFGNLIALSLGLTPNFKSNFDLAEDAKLQLSKDTYDDDLDNLLAQIGDQYADLFLAAKNLSDAILLSDILRVNTEITKAPLSASMIKRYDEHHQDLTLLKALVRQQLPEKYKEIFFDQSKNGYAGYIDGGASQEEFYKFIKPILEKMDGTEELLVKLNREDLLRKQRTFDNGSIPHQIHLGELHAILRRQEDFYPFLKDNREKIEKILTFRIPYYVGPLARGNSRFAWMTRKSEETITPWNFEEVVDKGASAQSFIERMTNFDKNLPNEKVLPKHSLLYEYFTVYNELTKVKYVTEGMRKPAFLSGEQKKAIVDLLFKTNRKVTVKQLKEDYFKKIECFDSVEISGVEDRFNASLGTYHDLLKIIKDKDFLDNEENEDILEDIVLTLTLFEDREMIEERLKTYAHLFDDKVMKQLKRRRYTGWGRLSRKLINGIRDKQSGKTILDFLKSDGFANRNFMQLIHDDSLTFKEDIQKAQVSGQGDSLHEHIANLAGSPAIKKGILQTVKVVDELVKVMGRHKPENIVIEMARENQTTQKGQKNSRERMKRIEEGIKELGSQILKEHPVENTQLQNEKLYLYYLQNGRDMYVDQELDINRLSDYDVDHIVPQSFLKDDSIDNKVLTRSDKNRGKSDNVPSEEVVKKMKNYWRQLLNAKLITQRKFDNLTKAERGGLSELDKAGFIKRQLVETRQITKHVAQILDSRMNTKYDENDKLIREVKVITLKSKLVSDFRKDFQFYKVREINNYHHAHDAYLNAVVGTALIKKYPKLESEFVYGDYKVYDVRKMIAKSEQEIGKATAKYFFYSNIMNFFKTEITLANGEIRKRPLIETNGETGEIVWDKGRDFATVRKVLSMPQVNIVKKTEVQTGGFSKESILPKRNSDKLIARKKDWDPKKYGGFDSPTVAYSVLVVAKVEKGKSKKLKSVKELLGITIMERSSFEKNPIDFLEAKGYKEVKKDLIIKLPKYSLFELENGRKRMLASAGELQKGNELALPSKYVNFLYLASHYEKLKGSPEDNEQKQLFVEQHKHYLDEIIEQISEFSKRVILADANLDKVLSAYNKHRDKPIREQAENIIHLFTLTNLGAPAAFKYFDTTIDRKRYTSTKEVLDATLIHQSITGLYETRIDLSQLGGD

SEQ ID NO: 19 - DNA, 4101 bp, Artificial Sequence
  Cas9 D10A Protein Nucleotide Sequence
gataaaaagtattctattggtttagccatcggcactaattccgttggatgggctgtcataaccgatgaatacaaagtaccttcaaagaaatttaaggtgttggggaacacagaccgtcattcgattaaaaagaatcttatcggtgccctcctattcgatagtggcgaaacggcagaggcgactcgcctgaaacgaaccgctcggagaaggtatacacgtcgcaagaaccgaatatgttacttacaagaaatttttagcaatgagatggccaaagttgacgattctttctttcaccgtttggaagagtccttccttgtcgaagaggacaagaaacatgaacggcaccccatctttggaaacatagtagatgaggtggcatatcatgaaaagtacccaacgatttatcacctcagaaaaaagctagttgactcaactgataaagcggacctgaggttaatctacttggctcttgcccatatgataaagttccgtgggcactttctcattgagggtgatctaaatccggacaactcggatgtcgacaaactgttcatccagttagtacaaacctataatcagttgtttgaagagaaccctataaatgcaagtggcgtggatgcgaaggctattcttagcgcccgcctctctaaatcccgacggctagaaaacctgatcgcacaattacccggagagaagaaaaatgggttgttcggtaaccttatagcgctctcactaggcctgacaccaaattttaagtcgaacttcgacttagctgaagatgccaaattgcagcttagtaaggacacgtacgatgacgatctcgacaatctactggcacaaattggagatcagtatgcggacttatttttggctgccaaaaaccttagcgatgcaatcctcctatctgacatactgagagttaatactgagattaccaaggcgccgttatccgcttcaatgatcaaaaggtacgatgaacatcaccaagacttgacacttctcaaggccctagtccgtcagcaactgcctgagaaatataaggaaatattctttgatcagtcgaaaaacgggtacgcaggttatattgacggcggagcgagtcaagaggaattctacaagtttatcaaacccatattagagaagatggatgggacggaagagttgcttgtaaaactcaatcgcgaagatctactgcgaaagcagcggactttcgacaacggtagcattccacatcaaatccacttaggcgaattgcatgctatacttagaaggcaggaggatttttatccgttcctcaaagacaatcgtgaaaagattgagaaaatcctaacctttcgcataccttactatgtgggacccctggcccgagggaactctcggttcgcatggatgacaagaaagtccgaagaaacgattactccatggaattttgaggaagttgtcgataaaggtgcgtcagctcaatcgttcatcgagaggatgaccaactttgacaagaatttaccgaacgaaaaagtattgcctaagcacagtttactttacgagtatttcacagtgtacaatgaactcacgaaagttaagtatgtcactgagggcatgcgtaaacccgcctttctaagcggagaacagaagaaagcaatagtagatctgttattcaagaccaaccgcaaagtgacagttaagcaattgaaagaggactactttaagaaaattgaatgcttcgattctgtcgagatctccggggtagaagatcgatttaatgcgtcacttggtacgtatcatgacctcctaaagataattaaagataaggacttcctggataacgaagagaatgaagatatcttagaagatatagtgttgactcttaccctctttgaagatcgggaaatgattgaggaaagactaaaaacatacgctcacctgttcgacgataaggttatgaaacagttaaagaggcgtcgctatacgggctggggacgattgtcgcggaaacttatcaacgggataagagacaagcaaagtggtaaaactattctcgattttctaaagagcgacggcttcgccaataggaactttatgcagctgatccatgatgactctttaaccttcaaagaggatatacaaaaggcacaggtttccggacaaggggactcattgcacgaacatattgcgaatcttgctggttcgccagccatcaaaaagggcatactccagacagtcaaagtagtggatgagctagttaaggtcatgggacgtcacaaaccggaaaacattgtaatcgagatggcacgcgaaaatcaaacgactcagaaggggcaaaaaaacagtcgagagcggatgaagagaatagaagagggtattaaagaactgggcagccagatcttaaaggagcatcctgtggaaaatacccaattgcagaacgagaaactttacctctattacctacaaaatggaagggacatgtatgttgatcaggaactggacataaaccgtttatctgattacgacgtcgatcacattgtaccccaatcctttttgaaggacgattcaatcgacaataaagtgcttacacgctcggataagaaccgagggaaaagtgacaatgttccaagcgaggaagtcgtaaagaaaatgaagaactattggcggcagctcctaaatgcgaaactgataacgcaaagaaagttcgataacttaactaaagctgagaggggtggcttgtctgaacttgacaaggccggatttattaaacgtcagctcgtggaaacccgccaaatcacaaagcatgttgcacagatactagattcccgaatgaatacgaaatacgacgagaacgataagctgattcgggaagtcaaagtaatcactttaaagtcaaaattggtgtcggacttcagaaaggattttcaattctataaagttagggagataaataactaccaccatgcgcacgacgcttatcttaatgccgtcgtagggaccgcactcattaagaaatacccgaagctagaaagtgagtttgtgtatggtgattacaaagtttatgacgtccgtaagatgatcgcgaaaagcgaacaggagataggcaaggctacagccaaatacttcttttattctaacattatgaatttctttaagacggaaatcactctggcaaacggagagatacgcaaacgacctttaattgaaaccaatggggagacaggtgaaatcgtatgggataagggccgggacttcgcgacggtgagaaaagttttgtccatgccccaagtcaacatagtaaagaaaactgaggtgcagaccggagggttttcaaaggaatcgattcttccaaaaaggaatagtgataagctcatcgctcgtaaaaaggactgggacccgaaaaagtacggtggcttcgatagccctacagttgcctattctgtcctagtagtggcaaaagttgagaagggaaaatccaagaaactgaagtcagtcaaagaattattggggataacgattatggagcgctcgtcttttgaaaagaaccccatcgacttccttgaggcgaaaggttacaaggaagtaaaaaaggatctcataattaaactaccaaagtatagtctgtttgagttagaaaatggccgaaaacggatgttggctagcgccggagagcttcaaaaggggaacgaactcgcactaccgtctaaatacgtgaatttcctgtatttagcgtcccattacgagaagttgaaaggttcacctgaagataacgaacagaagcaactttttgttgagcagcacaaacattatctcgacgaaatcatagagcaaatttcggaattcagtaagagagtcatcctagctgatgccaatctggacaaagtattaagcgcatacaacaagcacagggataaacccatacgtgagcaggcggaaaatattatccatttgtttactcttaccaacctcggcgctccagccgcattcaagtattttgacacaacgatagatcgcaaacgatacacttctaccaaggaggtgctagacgcgacactgattcaccaatccatcacgggattatatgaaactcggatagatttgtcacagcttgggggtgac

SEQ ID NO: 20 - DNA, 128 bp, Artificial Sequence
  RNA scaffold expression cassette (S. pyogenes), containing a 20-nucleotide programmable sequence, a CRISPR RNA motif, and an MS2 aptamer motif seq
  misc_feature (1)..(20): n is a, c, g, or t
nnnnnnnnnnnnnnnnnnnngttttagagctagaaatagcaagttaaaataaggctagtccgttatcaacttgaaaaagtggcaccgagtcggtgcgcgcacatgaggatcacccatgtgcttttttt

SEQ ID NO: 21 - DNA, 150 bp, Artificial Sequence
  RNA scaffold containing two MS2 loops seq
gttttagagctagaaatagcaagttaaaataaggctagtccgttatcaacttgaaaaagtggcaccgagtcggtgcgggagcacatgaggatcacccatgtgccacgagcgacatgaggatcacccatgtcgctcgtgttcccttttttt

SEQ ID NO: 22 - protein, 340 aa, Artificial Sequence
  Effector AID-MCP fusion
MDSLLMNRRKFLYQFKNVRWAKGRRETYLCYVVKRRDSATSFSLDFGYLRNKNGCHVELLFLRYISDWDLDPGRCYRVTWFTSWSPCYDCARHVADFLRGNPNLSLRIFTARLYFCEDRKAEPEGLRRLHRAGVQIAIMTFKDYFYCWNTFVENHERTFKAWEGLHENSVRLSRQLRRILLPLYEVDDLRDAFRTLGLELKTPLGDTTHTSPPCPAPELLGGPMASNFTQFVLVDNGGTGDVTVAPSNFANGIAEWISSNSRSQAYKVTCSVRQSSAQNRKYTIKVEVPKGAWRSYLNMELTIPIFATNSDCELIVKAMQGLLKDGNPIPSAIAANSGIY

SEQ ID NO: 23 - DNA, 594 bp, Artificial Sequence
  wtAID cDNA seq
atggacagcctcttgatgaaccggaggaagtttctttaccaattcaaaaatgtccgctgggctaagggtcggcgtgagacctacctgtgctacgtagtgaagaggcgtgacagtgctacatccttttcactggactttggttatcttcgcaataagaacggctgccacgtggaattgctcttcctccgctacatctcggactgggacctagaccctggccgctgctaccgcgtcacctggttcacctcctggagcccctgctacgactgtgcccgacatgtggccgactttctgcgagggaaccccaacctcagtctgaggatcttcaccgcgcgcctctacttctgtgaggaccgcaaggctgagcccgaggggctgcggcggctgcaccgcgccggggtgcaaatagccatcatgaccttcaaagattatttttactgctggaatacttttgtagaaaaccatgaaagaactttcaaagcctgggaagggctgcatgaaaattcagttcgtctctccagacagcttcggcgcatccttttgcccctgtatgaggttgatgacttacgagacgcatttcgtactttgggactt

SEQ ID NO: 24 - protein, 198 aa, Artificial Sequence [sequence omitted]

SEQ ID NO: 25 - DNA, 594 bp, Artificial Sequence
  AID_S38A cDNA seq
atggacagcctcttgatgaaccggaggaagtttctttaccaattcaaaaatgtccgctgggctaagggtcggcgtgagacctacctgtgctacgtagtgaagaggcgtgacgccgctacatccttttcactggactttggttatcttcgcaataagaacggctgccacgtggaattgctcttcctccgctacatctcggactgggacctagaccctggccgctgctaccgcgtcacctggttcacctcctggagcccctgctacgactgtgcccgacatgtggccgactttctgcgagggaaccccaacctcagtctgaggatcttcaccgcgcgcctctacttctgtgaggaccgcaaggctgagcccgaggggctgcggcggctgcaccgcgccggggtgcaaatagccatcatgaccttcaaagattatttttactgctggaatacttttgtagaaaaccatgaaagaactttcaaagcctgggaagggctgcatgaaaattcagttcgtctctccagacagcttcggcgcatccttttgcccctgtatgaggttgatgacttacgagacgcatttcgtactttgggactt

SEQ ID NO: 26 - protein, 198 aa, Artificial Sequence
  AID_S38A protein seq
MDSLLMNRRKFLYQFKNVRWAKGRRETYLCYVVKRRDAATSFSLDFGYLRNKNGCHVELLFLRYISDWDLDPGRCYRVTWFTSWSPCYDCARHVADFLRGNPNLSLRIFTARLYFCEDRKAEPEGLRRLHRAGVQIAIMTFKDYFYCWNTFVENHERTFKAWEGLHENSVRLSRQLRRILLPLYEVDDLRDAFRTLGL

SEQ ID NO: 27 - DNA, 624 bp, Artificial Sequence
  Humanised nucleotide sequence PmCDA1 (Petromyzon marinus)
atgaccgacgctgaatacgtcaggatacacgaaaagctcgatatttacacctttaagaaacagttcttcaataataagaagagtgtttcacatcgatgctatgtgcttttcgagctcaaacggcgaggagaaaggagagcatgtttttggggctacgctgtaaacaaaccccaatctggcacagagcggggcattcacgccgaaattttttccatcaggaaagtcgaggaatacttgcgcgataaccccggtcaatttacaatcaactggtattcttcatggtccccctgcgctgactgcgccgaaaagatcttggaatggtataaccaggaacttagaggtaacggtcacactctcaaaatatgggcctgcaaactttactacgagaagaatgctcgaaaccaaataggcctgtggaatcttcgcgataacggggtgggacttaatgtcatggtaagcgaacactaccaatgctgccgcaagatttttatacagtctagtcataaccagcttaacgagaaccgctggcttgaaaagacgctcaaacgggcggaaaaaaggaggagtgagctcagtataatgattcaagtgaaaatactgcacacgactaagtcaccagcagta

SEQ ID NO: 28 - protein, 208 aa, Artificial Sequence
  Amino acid sequence PmCDA1
MTDAEYVRIHEKLDIYTFKKQFFNNKKSVSHRCYVLFELKRRGERRACFWGYAVNKPQSGTERGIHAEIFSIRKVEEYLRDNPGQFTINWYSSWSPCADCAEKILEWYNQELRGNGHTLKIWACKLYYEKNARNQIGLWNLRDNGVGLNVMVSEHYQCCRKIFIQSSHNQLNENRWLEKTLKRAEKRRSELSIMIQVKILHTTKSPAV

SEQ ID NO: 29 - protein, 350 aa, Artificial Sequence
  PmCDA1-linker-MCP seq
MTDAEYVRIHEKLDIYTFKKQFFNNKKSVSHRCYVLFELKRRGERRACFWGYAVNKPQSGTERGIHAEIFSIRKVEEYLRDNPGQFTINWYSSWSPCADCAEKILEWYNQELRGNGHTLKIWACKLYYEKNARNQIGLWNLRDNGVGLNVMVSEHYQCCRKIFIQSSHNQLNENRWLEKTLKRAEKRRSELSIMIQVKILHTTKSPAVELKTPLGDTTHTSPPCPAPELLGGPMASNFTQFVLVDNGGTGDVTVAPSNFANGIAEWISSNSRSQAYKVTCSVRQSSAQNRKYTIKVEVPKGAWRSYLNMELTIPIFATNSDCELIVKAMQGLLKDGNPIPSAIAANSGIY

SEQ ID NO: 30 - RNA, 135 nt, Artificial Sequence
  Sequence of gRNA_MS2 construct
  misc_feature (1)..(20): n is a, c, g, or u
nnnnnnnnnnnnnnnnnnnnguuuuagagcuaugcuguugaaaaacagcauagcaaguuaaaauaaggcuaguccguuaucaacuugaaaaaguggcaccgagucggugcgcgcacaugaggaucacccaugugc

SEQ ID NO: 31 - RNA, 149 nt, Artificial Sequence
  Sequence of gRNA_2xMS2 construct
  misc_feature (1)..(19): n is a, c, g, or u
nnnnnnnnnnnnnnnnnnnguuuuagagcuagaaauagcaaguuaaaauaaggcuaguccguuaucaacuugaaaaaguggcaccgagucggugcgggagcacaugaggaucacccaugugccacgagcgacaugaggaucacccaugu

SEQ ID NO: 32 - DNA, 42 bp, Artificial Sequence
  Synthetic crRNA Sequence
  m (1)..(2): 2'Oxymethyl
  Phosphorothioate-bonds (1)..(3): Phosphorothioate bonds between bases 1&2, 2&3
cacctacctaagaaccatccguuuuagagcuaugcuguuuug

SEQ ID NO: 33 - RNA, 99 nt, Artificial Sequence; identical to SEQ ID NO: 2
  Synthetic tracrRNA-MS2 Aptamer Sequence
  m (97)..(98): 2'Oxymethyl modification
  Phosphorothioate-bonds (97)..(99): Phosphorothioate bonds between bases 97&98, 98&99

SEQ ID NO: 34 - RNA, 128 nt, Artificial Sequence
  B2M sgRNA seq
  m (1)..(2): 2'Oxymethyl modification
  Phosphorothioate-bonds (1)..(3): Phosphorothioate bonds between bases 1&2, 2&3
  m (126)..(127): 2'Oxymethyl modification
  Phosphorothioate-bonds (126)..(128): Phosphorothioate bonds between bases 126&127, 127&128
uucguaucuguaaaaccaagguuuuagagcuagaaauagcaaguuaaaauaaggcuaguccguuaucaacuugaaaaaguggcaccgagucggugcgcgcacaugaggaucacccaugugcuuuuuuu

SEQ ID NO: 35 - RNA, 128 nt, Artificial Sequence
  CD52 sgRNA seq
  m (1)..(2): 2'Oxymethyl modification
  Phosphorothioate-bonds (1)..(3): Phosphorothioate bonds between bases 1&2, 2&3
  m (126)..(127): 2'Oxymethyl modification
  Phosphorothioate-bonds (126)..(128): Phosphorothioate bonds between bases 126&127, 127&128
acucacgcuggauagccuccguuuuagagcuagaaauagcaaguuaaaauaaggcuaguccguuaucaacuugaaaaaguggcaccgagucggugcgcgcacaugaggaucacccaugugcuuuuuuu

SEQ ID NO: 36 - RNA, 128 nt, Artificial Sequence
  TRAC sgRNA seq
  m (1)..(2): 2'Oxymethyl modification
  Phosphorothioate-bonds (1)..(3): Phosphorothioate bonds between bases 1&2, 2&3
  m (126)..(127): 2'Oxymethyl modification
  Phosphorothioate-bonds (126)..(128): Phosphorothioate bonds between bases 126&127, 127&128
cucuuaccuguaccauaaccguuuuagagcuagaaauagcaaguuaaaauaaggcuaguccguuaucaacuugaaaaaguggcaccgagucggugcgcgcacaugaggaucacccaugugcuuuuuuu

SEQ ID NO: 37 - RNA, 128 nt, Artificial Sequence
  PDCD-1 sgRNA seq
  m (1)..(2): 2'Oxymethyl modification
  Phosphorothioate-bonds (1)..(3): Phosphorothioate bonds between bases 1&2, 2&3
  m (126)..(127): 2'Oxymethyl modification
  Phosphorothioate-bonds (126)..(128): Phosphorothioate bonds between bases 126&127, 127&128
caccuaccuaagaaccauccguuuuagagcuagaaauagcaaguuaaaauaaggcuaguccguuaucaacuugaaaaaguggcaccgagucggugcgcgcacaugaggaucacccaugugcuuuuuuu

SEQ ID NO: 38 - RNA, 128 nt, Artificial Sequence
  Scramble sgRNA seq
  m (1)..(2): 2'Oxymethyl modification
  Phosphorothioate-bonds (1)..(3): Phosphorothioate bonds between bases 1&2, 2&3
  m (126)..(127): 2'Oxymethyl modification
  Phosphorothioate-bonds (126)..(128): Phosphorothioate bonds between bases 126&127, 127&128
gcacuaccagagcuaacucaguuuuagagcuagaaauagcaaguuaaaauaaggcuaguccguuaucaacuugaaaaaguggcaccgagucggugcgcgcacaugaggaucacccaugugcuuuuuuu

SEQ ID NO: 39 - protein, 319 aa, Artificial Sequence
  NLS-Anolis(P16A-E17A)-Apobec1-Linker-MCP seq
MAPKKKRKVMEPEAFQRNFDPREFAACTLLLYEIHWDNNTSRNWCTNKPGLHAEENFLQIFNEKIDIKQDTPCSITWFLSWSPCYPCSQAIIKFLEAHPNVSLEIKAARLYMHQIDCNKEGLRNLGRNRVSIMNLPDYRHCWTTFVVPRGANEDYWPQDFLPAITNYSRELDSILQDELKTPLGDTTHTSPPCPAPELLGGPMASNFTQFVLVDNGGTGDVTVAPSNFANGIAEWISSNSRSQAYKVTCSVRQSSAQNRKYTIKVEVPKGAWRSYLNMELTIPIFATNSDCELIVKAMQGLLKDGNPIPSAIAANSGIY

SEQ ID NO: 40 - protein, 379 aa, Artificial Sequence
  NLS-Rattus-Apobec1-Linker-MCP seq
MAPKKKRKVSSETGPVAVDPTLRRRIEPHEFEVFFDPRELRKETCLLYEINWGGRHSIWRHTSQNTNKHVEVNFIEKFTTERYFCPNTRCSITWFLSWSPCGECSRAITEFLSRYPHVTLFIYIARLYHHADPRNRQGLRDLISSGVTIQIMTEQESGYCWRNFVNYSPSNEAHWPRYPHLWVRLYVLELYCIILGLPPCLNILRRKQPQLTFFTIALQSCHYQRLPPHILWATGLKELKTPLGDTTHTSPPCPAPELLGGPMASNFTQFVLVDNGGTGDVTVAPSNFANGIAEWISSNSRSQAYKVTCSVRQSSAQNRKYTIKVEVPKGAWRSYLNMELTIPIFATNSDCELIVKAMQGLLKDGNPIPSAIAANSGIY

SEQ ID NO: 41 - protein, 349 aa, Artificial Sequence
  NLS-Homo-AID-L25-MCP seq
MAPKKKRKVMDSLLMNRRKFLYQFKNVRWAKGRRETYLCYVVKRRDSATSFSLDFGYLRNKNGCHVELLFLRYISDWDLDPGRCYRVTWFTSWSPCYDCARHVADFLRGNPNLSLRIFTARLYFCEDRKAEPEGLRRLHRAGVQIAIMTFKDYFYCWNTFVENHERTFKAWEGLHENSVRLSRQLRRILLPLYEVDDLRDAFRTLGLELKTPLGDTTHTSPPCPAPELLGGPMASNFTQFVLVDNGGTGDVTVAPSNFANGIAEWISSNSRSQAYKVTCSVRQSSAQNRKYTIKVEVPKGAWRSYLNMELTIPIFATNSDCELIVKAMQGLLKDGNPIPSAIAANSGIY

SEQ ID NO: 42 - protein, 1582 aa, Artificial Sequence
  NLS-nCas9(D10A)-UGI-UGI-NLS seq
MPKKKRKVDKKYSIGLAIGTNSVGWAVITDEYKVPSKKFKVLGNTDRHSIKKNLIGALLFDSGETAEATRLKRTARRRYTRRKNRICYLQEIFSNEMAKVDDSFFHRLEESFLVEEDKKHERHPIFGNIVDEVAYHEKYPTIYHLRKKLVDSTDKADLRLIYLALAHMIKFRGHFLIEGDLNPDNSDVDKLFIQLVQTYNQLFEENPINASGVDAKAILSARLSKSRRLENLIAQLPGEKKNGLFGNLIALSLGLTPNFKSNFDLAEDAKLQLSKDTYDDDLDNLLAQIGDQYADLFLAAKNLSDAILLSDILRVNTEITKAPLSASMIKRYDEHHQDLTLLKALVRQQLPEKYKEIFFDQSKNGYAGYIDGGASQEEFYKFIKPILEKMDGTEELLVKLNREDLLRKQRTFDNGSIPHQIHLGELHAILRRQEDFYPFLKDNREKIEKILTFRIPYYVGPLARGNSRFAWMTRKSEETITPWNFEEVVDKGASAQSFIERMTNFDKNLPNEKVLPKHSLLYEYFTVYNELTKVKYVTEGMRKPAFLSGEQKKAIVDLLFKTNRKVTVKQLKEDYFKKIECFDSVEISGVEDRFNASLGTYHDLLKIIKDKDFLDNEENEDILEDIVLTLTLFEDREMIEERLKTYAHLFDDKVMKQLKRRRYTGWGRLSRKLINGIRDKQSGKTILDFLKSDGFANRNFMQLIHDDSLTFKEDIQKAQVSGQGDSLHEHIANLAGSPAIKKGILQTVKVVDELVKVMGRHKPENIVIEMARENQTTQKGQKNSRERMKRIEEGIKELGSQILKEHPVENTQLQNEKLYLYYLQNGRDMYVDQELDINRLSDYDVDHIVPQSFLKDDSIDNKVLTRSDKNRGKSDNVPSEEVVKKMKNYWRQLLNAKLITQRKFDNLTKAERGGLSELDKAGFIKRQLVETRQITKHVAQILDSRMNTKYDENDKLIREVKVITLKSKLVSDFRKDFQFYKVREINNYHHAHDAYLNAVVGTALIKKYPKLESEFVYGDYKVYDVRKMIAKSEQEIGKATAKYFFYSNIMNFFKTEITLANGEIRKRPLIETNGETGEIVWDKGRDFATVRKVLSMPQVNIVKKTEVQTGGFSKESILPKRNSDKLIARKKDWDPKKYGGFDSPTVAYSVLVVAKVEKGKSKKLKSVKELLGITIMERSSFEKNPIDFLEAKGYKEVKKDLIIKLPKYSLFELENGRKRMLASAGELQKGNELALPSKYVNFLYLASHYEKLKGSPEDNEQKQLFVEQHKHYLDEIIEQISEFSKRVILADANLDKVLSAYNKHRDKPIREQAENIIHLFTLTNLGAPAAFKYFDTTIDRKRYTSTKEVLDATLIHQSITGLYETRIDLSQLGGDSGGSGGSGGSTNLSDIIEKETGKQLVIQESILMLPEEVEEVIGNKPESDILVHTAYDESTDENVMLLTSDAPEYKPWALVIQDSNGENKIKMLSGGSGGSGGSTNLSDIIEKETGKQLVIQESILMLPEEVEEVIGNKPESDILVHTAYDESTDENVMLLTSDAPEYKPWALVIQDSNGENKIKMLSGGSKRTADGSEFEPKKKRKV

SEQ ID NO: 43 - DNA, 4104 bp, Artificial Sequence
  Humanised nucleotide sequence WT Streptococcus pyogenes Cas9
atggacaagaagtacagcatcggcctggacatcggcaccaactctgtgggctgggccgtgatcaccgacgagtacaaggtgcccagcaagaaattcaaggtgctgggcaacaccgaccggcacagcatcaagaagaacctgatcggagccctgctgttcgacagcggcgaaacagccgaggccacccggctgaagagaaccgccagaagaagatacaccagacggaagaaccggatctgctatctgcaagagatcttcagcaacgagatggccaaggtggacgacagcttcttccacagactggaagagtccttcctggtggaagaggataagaagcacgagcggcaccccatcttcggcaacatcgtggacgaggtggcctaccacgagaagtaccccaccatctaccacctgagaaagaaactggtggacagcaccgacaaggccgacctgcggctgatctatctggccctggcccacatgatcaagttccggggccacttcctgatcgagggcgacctgaaccccgacaacagcgacgtggacaagctgttcatccagctggtgcagacctacaaccagctgttcgaggaaaaccccatcaacgccagcggcgtggacgccaaggccatcctgtctgccagactgagcaagagcagacggctggaaaatctgatcgcccagctgcccggcgagaagaagaatggcctgttcggaaacctgattgccctgagcctgggcctgacccccaacttcaagagcaacttcgacctggccgaggatgccaaactgcagctgagcaaggacacctacgacgacgacctggacaacctgctggcccagatcggcgaccagtacgccgacctgtttctggccgccaagaacctgtccgacgccatcctgctgagcgacatcctgagagtgaacaccgagatcaccaaggcccccctgagcgcctctatgatcaagagatacgacgagcaccaccaggacctgaccctgctgaaagctctcgtgcggcagcagctgcctgagaagtacaaagagattttcttcgaccagagcaagaacggctacgccggctacattgacggcggagccagccaggaagagttctacaagttcatcaagcccatcctggaaaagatggacggcaccgaggaactgctcgtgaagctgaacagagaggacctgctgcggaagcagcggaccttcgacaacggcagcatcccccaccagatccacctgggagagctgcacgccattctgcggcggcaggaagatttttacccattcctgaaggacaaccgggaaaagatcgagaagatcctgaccttccgcatcccctactacgtgggccctctggccaggggaaacagcagattcgcctggatgaccagaaagagcgaggaaaccatcaccccctggaacttcgaggaagtggtggacaagggcgcttccgcccagagcttcatcgagcggatgaccaacttcgataagaacctgcccaacgagaaggtgctgcccaagcacagcctgctgtacgagtacttcaccgtgtataacgagctgaccaaagtgaaatacgtgaccgagggaatgagaaagcccgccttcctgagcggcgagcagaaaaaggccatcgtggacctgctgttcaagaccaaccggaaagtgaccgtgaagcagctgaaagaggactacttcaagaaaatcgagtgcttcgactccgtggaaatctccggcgtggaagatcggttcaacgcctccctgggcacataccacgatctgctgaaaattatcaaggacaaggacttcctggacaatgaggaaaacgaggacattctggaagatatcgtgctgaccctgacactgtttgaggacagagagatgatcgaggaacggctgaaaacctatgcccacctgttcgacgacaaagtgatgaagcagctgaagcggcggagatacaccggctggggcaggctgagccggaagctgatcaacggcatccgggacaagcagtccggcaagacaatcctggatttcctgaagtccgacggcttcgccaacagaaacttcatgcagctgatccacgacgacagcctgacctttaaagaggacatccagaaagcccaggtgtccggccagggcgatagcctgcacgagcacattgccaatctggccggcagccccgccattaagaagggcatcctgcagacagtgaaggtggtggacgagctcgtgaaagtgatgggccggcacaagcccgagaacatcgtgatcgaaatggccagagagaaccagaccacccagaagggacagaagaacagccgcgagagaatgaagcggatcgaagagggcatcaaagagctgggcagccagatcctgaaagaacaccccgtggaaaacacccagctgcagaacgagaagctgtacctgtactacctgcagaatgggcgggatatgtacgtggaccaggaactggacatcaaccggctgtccgactacgatgtggaccatatcgtgcctcagagctttctgaaggacgactccatcgacaacaaggtgctgaccagaagcgacaagaaccggggcaagagcgacaacgtgccctccgaagaggtcgtgaagaagatgaagaactactggcggcagctgctgaacgccaagctgattacccagagaaagttcgacaatctgaccaaggccgagagaggcggcctgagcgaactggataaggccggcttcatcaagagacagctggtggaaacccggcagatcacaaagcacgtggcacagatcctggactcccggatgaacactaagtacgacgagaatgacaagctgatccgggaagtgaaagtgatcaccctgaagtccaagctggtgtccgatttccggaaggatttccagttttacaaagtgcgcgagatcaacaactaccaccacgcccacgacgcctacctgaacgccgtcgtgggaaccgccctgatcaaaaagtaccctaagctggaaagcgagttcgtgtacggcgactacaaggtgtacgacgtgcggaagatgatcgccaagagcgagcaggaaatcggcaaggctaccgccaagtacttcttctacagcaacatcatgaactttttcaagaccgagattaccctggccaacggcgagatccggaagcggcctctgatcgagacaaacggcgaaaccggggagatcgtgtgggataagggccgggattttgccaccgtgcggaaagtgctgagcatgccccaagtgaatatcgtgaaaaagaccgaggtgcagacaggcggcttcagcaaagagtctatcctgcccaagaggaacagcgataagctgatcgccagaaagaaggactgggaccctaagaagtacggcggcttcgacagccccaccgtggcctattctgtgctggtggtggccaaagtggaaaagggcaagtccaagaaactgaagagtgtgaaagagctgctggggatcaccatcatggaaagaagcagcttcgagaagaatcccatcgactttctggaagccaagggctacaaagaagtgaaaaaggacctgatcatcaagctgcctaagtactccctgttcgagctggaaaacggccggaagagaatgctggcctctgccggcgaactgcagaagggaaacgaactggccctgccctccaaatatgtgaacttcctgtacctggccagccactatgagaagctgaagggctcccccgaggataatgagcagaaacagctgtttgtggaacagcacaagcactacctggacgagatcatcgagcagatcagcgagttctccaagagagtgatcctggccgacgctaatctggacaaagtgctgtccgcctacaacaagcaccgggataagcccatcagagagcaggccgagaatatcatccacctgtttaccctgaccaatctgggagcccctgccgccttcaagtactttgacaccaccatcgaccggaagaggtacaccagcaccaaagaggtgctggacgccaccctgatccaccagagcatcaccggcctgtacgagacacggatcgacctgtctcagctgggaggtgac

SEQ ID NO: 44 - protein, 1368 aa, Artificial Sequence [sequence omitted]

SEQ ID NO: 45 - DNA, 4104 bp, Artificial Sequence
  Humanised nucleotide sequence Streptococcus pyogenes nCas9
atggacaagaagtacagcatcggcctggccatcggcaccaactctgtgggctgggccgtgatcaccgacgagtacaaggtgcccagcaagaaattcaaggtgctgggcaacaccgaccggcacagcatcaagaagaacctgatcggagccctgctgttcgacagcggcgaaacagccgaggccacccggctgaagagaaccgccagaagaagatacaccagacggaagaaccggatctgctatctgcaagagatcttcagcaacgagatggccaaggtggacgacagcttcttccacagactggaagagtccttcctggtggaagaggataagaagcacgagcggcaccccatcttcggcaacatcgtggacgaggtggcctaccacgagaagtaccccaccatctaccacctgagaaagaaactggtggacagcaccgacaaggccgacctgcggctgatctatctggccctggcccacatgatcaagttccggggccacttcctgatcgagggcgacctgaaccccgacaacagcgacgtggacaagctgttcatccagctggtgcagacctacaaccagctgttcgaggaaaaccccatcaacgccagcggcgtggacgccaaggccatcctgtctgccagactgagcaagagcagacggctggaaaatctgatcgcccagctgcccggcgagaagaagaatggcctgttcggaaacctgattgccctgagcctgggcctgacccccaacttcaagagcaacttcgacctggccgaggatgccaaactgcagctgagcaaggacacctacgacgacgacctggacaacctgctggcccagatcggcgaccagtacgccgacctgtttctggccgccaagaacctgtccgacgccatcctgctgagcgacatcctgagagtgaacaccgagatcaccaaggcccccctgagcgcctctatgatcaagagatacgacgagcaccaccaggacctgaccctgctgaaagctctcgtgcggcagcagctgcctgagaagtacaaagagattttcttcgaccagagcaagaacggctacgccggctacattgacggcggagccagccaggaagagttctacaagttcatcaagcccatcctggaaaagatggacggcaccgaggaactgctcgtgaagctgaacagagaggacctgctgcggaagcagcggaccttcgacaacggcagcatcccccaccagatccacctgggagagctgcacgccattctgcggcggcaggaagatttttacccattcctgaaggacaaccgggaaaagatcgagaagatcctgaccttccgcatcccctactacgtgggccctctggccaggggaaacagcagattcgcctggatgaccagaaagagcgaggaaaccatcaccccctggaacttcgaggaagtggtggacaagggcgcttccgcccagagcttcatcgagcggatgaccaacttcgataagaacctgcccaacgagaaggtgctgcccaagcacagcctgctgtacgagtacttcaccgtgtataacgagctgaccaaagtgaaatacgtgaccgagggaatgagaaagcccgccttcctgagcggcgagcagaaaaaggccatcgtggacctgctgttcaagaccaaccggaaagtgaccgtgaagcagctgaaagaggactacttcaagaaaatcgagtgcttcgactccgtggaaatctccggcgtggaagatcggttcaacgcctccctgggcacataccacgatctgctgaaaattatcaaggacaaggacttcctggacaatgaggaaaacgaggacattctggaagatatcgtgctgaccctgacactgtttgaggacagagagatgatcgaggaacggctgaaaacctatgcccacctgttcgacgacaaagtgatgaagcagctgaagcggcggagatacaccggctggggcaggctgagccggaagctgatcaacggcatccgggacaagcagtccggcaagacaatcctggatttcctgaagtccgacggcttcgccaacagaaacttcatgcagctgatccacgacgacagcctgacctttaaagaggacatccagaaagcccaggtgtccggccagggcgatagcctgcacgagcacattgccaatctggccggcagccccgccattaagaagggcatcctgcagacagtgaaggtggtggacgagctcgtgaaagtgatgggccggcacaagcccgagaacatcgtgatcgaaatggccagagagaaccagaccacccagaagggacagaagaacagccgcgagagaatgaagcggatcgaagagggcatcaaagagctgggcagccagatcctgaaagaacaccccgtggaaaacacccagctgcagaacgagaagctgtacctgtactacctgcagaatgggcgggatatgtacgtggaccaggaactggacatcaaccggctgtccgactacgatgtggaccatatcgtgcctcagagctttctgaaggacgactccatcgacaacaaggtgctgaccagaagcgacaagaaccggggcaagagcgacaacgtgccctccgaagaggtcgtgaagaagatgaagaactactggcggcagctgctgaacgccaagctgattacccagagaaagttcgacaatctgaccaaggccgagagaggcggcctgagcgaactggataaggccggcttcatcaagagacagctggtggaaacccggcagatcacaaagcacgtggcacagatcctggactcccggatgaacactaagtacgacgagaatgacaagctgatccgggaagtgaaagtgatcaccctgaagtccaagctggtgtccgatttccggaaggatttccagttttacaaagtgcgcgagatcaacaactaccaccacgcccacgacgcctacctgaacgccgtcgtgggaaccgccctgatcaaaaagtaccctaagctggaaagcgagttcgtgtacggcgactacaaggtgtacgacgtgcggaagatgatcgccaagagcgagcaggaaatcggcaaggctaccgccaagtacttcttctacagcaacatcatgaactttttcaagaccgagattaccctggccaacggcgagatccggaagcggcctctgatcgagacaaacggcgaaaccggggagatcgtgtgggataagggccgggattttgccaccgtgcggaaagtgctgagcatgccccaagtgaatatcgtgaaaaagaccgaggtgcagacaggcggcttcagcaaagagtctatcctgcccaagaggaacagcgataagctgatcgccagaaagaaggactgggaccctaagaagtacggcggcttcgacagccccaccgtggcctattctgtgctggtggtggccaaagtggaaaagggcaagtccaagaaactgaagagtgtgaaagagctgctggggatcaccatcatggaaagaagcagcttcgagaagaatcccatcgactttctggaagccaagggctacaaagaagtgaaaaaggacctgatcatcaagctgcctaagtactccctgttcgagctggaaaacggccggaagagaatgctggcctctgccggcgaactgcagaagggaaacgaactggccctgccctccaaatatgtgaacttcctgtacctggccagccactatgagaagctgaagggctcccccgaggataatgagcagaaacagctgtttgtggaacagcacaagcactacctggacgagatcatcgagcagatcagcgagttctccaagagagtgatcctggccgacgctaatctggacaaagtgctgtccgcctacaacaagcaccgggataagcccatcagagagcaggccgagaatatcatccacctgtttaccctgaccaatctgggagcccctgccgccttcaagtactttgacaccaccatcgaccggaagaggtacaccagcaccaaagaggtgctggacgccaccctgatccaccagagcatcaccggcctgtacgagacacggatcgacctgtctcagctgggaggtgac

SEQ ID NO: 46 - protein, 1368 aa, Artificial Sequence
  Humanised amino acid sequence Streptococcus pyogenes nCas9
MDKKYSIGLAIGTNSVGWAVITDEYKVPSKKFKVLGNTDRHSIKKNLIGALLFDSGETAEATRLKRTARRRYTRRKNRICYLQEIFSNEMAKVDDSFFHRLEESFLVEEDKKHERHPIFGNIVDEVAYHEKYPTIYHLRKKLVDSTDKADLRLIYLALAHMIKFRGHFLIEGDLNPDNSDVDKLFIQLVQTYNQLFEENPINASGVDAKAILSARLSKSRRLENLIAQLPGEKKNGLFGNLIALSLGLTPNFKSNFDLAEDAKLQLSKDTYDDDLDNLLAQIGDQYADLFLAAKNLSDAILLSDILRVNTEITKAPLSASMIKRYDEHHQDLTLLKALVRQQLPEKYKEIFFDQSKNGYAGYIDGGASQEEFYKFIKPILEKMDGTEELLVKLNREDLLRKQRTFDNGSIPHQIHLGELHAILRRQEDFYPFLKDNREKIEKILTFRIPYYVGPLARGNSRFAWMTRKSEETITPWNFEEVVDKGASAQSFIERMTNFDKNLPNEKVLPKHSLLYEYFTVYNELTKVKYVTEGMRKPAFLSGEQKKAIVDLLFKTNRKVTVKQLKEDYFKKIECFDSVEISGVEDRFNASLGTYHDLLKIIKDKDFLDNEENEDILEDIVLTLTLFEDREMIEERLKTYAHLFDDKVMKQLKRRRYTGWGRLSRKLINGIRDKQSGKTILDFLKSDGFANRNFMQLIHDDSLTFKEDIQKAQVSGQGDSLHEHIANLAGSPAIKKGILQTVKVVDELVKVMGRHKPENIVIEMARENQTTQKGQKNSRERMKRIEEGIKELGSQILKEHPVENTQLQNEKLYLYYLQNGRDMYVDQELDINRLSDYDVDHIVPQSFLKDDSIDNKVLTRSDKNRGKSDNVPSEEVVKKMKNYWRQLLNAKLITQRKFDNLTKAERGGLSELDKAGFIKRQLVETRQITKHVAQILDSRMNTKYDENDKLIREVKVITLKSKLVSDFRKDFQFYKVREINNYHHAHDAYLNAVVGTALIKKYPKLESEFVYGDYKVYDVRKMIAKSEQEIGKATAKYFFYSNIMNFFKTEITLANGEIRKRPLIETNGETGEIVWDKGRDFATVRKVLSMPQVNIVKKTEVQTGGFSKESILPKRNSDKLIARKKDWDPKKYGGFDSPTVAYSVLVVAKVEKGKSKKLKSVKELLGITIMERSSFEKNPIDFLEAKGYKEVKKDLIIKLPKYSLFELENGRKRMLASAGELQKGNELALPSKYVNFLYLASHYEKLKGSPEDNEQKQLFVEQHKHYLDEIIEQISEFSKRVILADANLDKVLSAYNKHRDKPIREQAENIIHLFTLTNLGAPAAFKYFDTTIDRKRYTSTKEVLDATLIHQSITGLYETRIDLSQLGGD

SEQ ID NO: 47 - DNA, 4104 bp, Artificial Sequence
  Humanised nucleotide sequence Streptococcus pyogenes dCas9
atggacaagaagtacagcatcggcctggccatcggcaccaactctgtgggctgggccgtgatcaccgacgagtacaaggtgcccagcaagaaattcaaggtgctgggcaacaccgaccggcacagcatcaagaagaacctgatcggagccctgctgttcgacagcggcgaaacagccgaggccacccggctgaagagaaccgccagaagaagatacaccagacggaagaaccggatctgctatctgcaagagatcttcagcaacgagatggccaaggtggacgacagcttcttccacagactggaagagtccttcctggtggaagaggataagaagcacgagcggcaccccatcttcggcaacatcgtggacgaggtggcctaccacgagaagtaccccaccatctaccacctgagaaagaaactggtggacagcaccgacaaggccgacctgcggctgatctatctggccctggcccacatgatcaagttccggggccacttcctgatcgagggcgacctgaaccccgacaacagcgacgtggacaagctgttcatccagctggtgcagacctacaaccagctgttcgaggaaaaccccatcaacgccagcggcgtggacgccaaggccatcctgtctgccagactgagcaagagcagacggctggaaaatctgatcgcccagctgcccggcgagaagaagaatggcctgttcggaaacctgattgccctgagcctgggcctgacccccaacttcaagagcaacttcgacctggccgaggatgccaaactgcagctgagcaaggacacctacgacgacgacctggacaacctgctggcccagatcggcgaccagtacgccgacctgtttctggccgccaagaacctgtccgacgccatcctgctgagcgacatcctgagagtgaacaccgagatcaccaaggcccccctgagcgcctctatgatcaagagatacgacgagcaccaccaggacctgaccctgctgaaagctctcgtgcggcagcagctgcctgagaagtacaaagagattttcttcgaccagagcaagaacggctacgccggctacattgacggcggagccagccaggaagagttctacaagttcatcaagcccatcctggaaaagatggacggcaccgaggaactgctcgtgaagctgaacagagaggacctgctgcggaagcagcggaccttcgacaacggcagcatcccccaccagatccacctgggagagctgcacgccattctgcggcggcaggaagatttttacccattcctgaaggacaaccgggaaaagatcgagaagatcctgaccttccgcatcccctactacgtgggccctctggccaggggaaacagcagattcgcctggatgaccagaaagagcgaggaaaccatcaccccctggaacttcgaggaagtggtggacaagggcgcttccgcccagagcttcatcgagcggatgaccaacttcgataagaacctgcccaacgagaaggtgctgcccaagcacagcctgctgtacgagtacttcaccgtgtataacgagctgaccaaagtgaaatacgtgaccgagggaatgagaaagcccgccttcctgagcggcgagcagaaaaaggccatcgtggacctgctgttcaagaccaaccggaaagtgaccgtgaagcagctgaaagaggactacttcaagaaaatcgagtgcttcgactccgtggaaatctccggcgtggaagatcggttcaacgcctccctgggcacataccacgatctgctgaaaattatcaaggacaaggacttcctggacaatgaggaaaacgaggacattctggaagatatcgtgctgaccctgacactgtttgaggacagagagatgatcgaggaacggctgaaaacctatgcccacctgttcgacgacaaagtgatgaagcagctgaagcggcggagatacaccggctggggcaggctgagccggaagctgatcaacggcatccgggacaagcagtccggcaagacaatcctggatttcctgaagtccgacggcttcgccaacagaaacttcatgcagctgatccacgacgacagcctgacctttaaagaggacatccagaaagcccaggtgtccggccagggcgatagcctgcacgagcacattgccaatctggccggcagccccgccattaagaagggcatcctgcagacagtgaaggtggtggacgagctcgtgaaagtgatgggccggcacaagcccgagaacatcgtgatcgaaatggccagagagaaccagaccacccagaagggacagaagaacagccgcgagagaatgaagcggatcgaagagggcatcaaagagctgggcagccagatcctgaaagaacaccccgtggaaaacacccagctgcagaacgagaagctgtacctgtactacctgcagaatgggcgggatatgtacgtggaccaggaactggacatcaaccggctgtccgactacgatgtggacgctatcgtgcctcagagctttctgaaggacgactccatcgacaacaaggtgctgaccagaagcgacaagaaccggggcaagagcgacaacgtgccctccgaagaggtcgtgaagaagatgaagaactactggcggcagctgctgaacgccaagctgattacccagagaaagttcgacaatctgaccaaggccgagagaggcggcctgagcgaactggataaggccggcttcatcaagagacagctggtggaaacccggcagatcacaaagcacgtggcacagatcctggactcccggatgaacactaagtacgacgagaatgacaagctgatccgggaagtgaaagtgatcaccctgaagtccaagctggtgtccgatttccggaaggatttccagttttacaaagtgcgcgagatcaacaactaccaccacgcccacgacgcctacctgaacgccgtcgtgggaaccgccctgatcaaaaagtaccctaagctggaaagcgagttcgtgtacggcgactacaaggtgtacgacgtgcggaagatgatcgccaagagcgagcaggaaatcggcaaggctaccgccaagtacttcttctacagcaacatcatgaactttttcaagaccgagattaccctggccaacggcgagatccggaagcggcctctgatcgagacaaacggcgaaaccggggagatcgtgtgggataagggccgggattttgccaccgtgcggaaagtgctgagcatgccccaagtgaatatcgtgaaaaagaccgaggtgcagacaggcggcttcagcaaagagtctatcctgcccaagaggaacagcgataagctgatcgccagaaagaaggactgggaccctaagaagtacggcggcttcgacagccccaccgtggcctattctgtgctggtggtggccaaagtggaaaagggcaagtccaagaaactgaagagtgtgaaagagctgctggggatcaccatcatggaaagaagcagcttcgagaagaatcccatcgactttctggaagccaagggctacaaagaagtgaaaaaggacctgatcatcaagctgcctaagtactccctgttcgagctggaaaacggccggaagagaatgctggcctctgccggcgaactgcagaagggaaacgaactggccctgccctccaaatatgtgaacttcctgtacctggccagccactatgagaagctgaagggctcccccgaggataatgagcagaaacagctgtttgtggaacagcacaagcactacctggacgagatcatcgagcagatcagcgagttctccaagagagtgatcctggccgacgctaatctggacaaagtgctgtccgcctacaacaagcaccgggataagcccatcagagagcaggccgagaatatcatccacctgtttaccctgaccaatctgggagcccctgccgccttcaagtactttgacaccaccatcgaccggaagaggtacaccagcaccaaagaggtgctggacgccaccctgatccaccagagcatcaccggcctgtacgagacacggatcgacctgtctcagctgggaggtgac

SEQ ID NO: 48 - protein, 1229 aa, Artificial Sequence
  Amino acid sequence WT AsCas12a
AIDSYRKEKTEETRNALIEEQATYRNAIHDYFIGRTDNLTDAINKRHAEIYKGLFKAELFNGKVLKQLGTVTTTEHENALLRSFDKFTTYFSGFYENRKNVFSAEDISTAIPHRIVQDNFPKFKENCHIFTRLITAVPSLREHFENVKKAIGIFVSTSIEEVFSFPFYNQLLTQTQIDLYNQLLGGISREAGTEKIKGLNEVLNLAIQKNDETAHIIASLPHRFIPLFKQILSDRNTLSFILEEFKSDEEVIQSFCKYKTLLRNENVLETAEALFNELNSIDLTHIFISHKKLETISSALCDHWDTLRNALYERRISELTGKITKSAKEKVQRSLKHEDINLQEIISAAGKELSEAFKQKTSEILSHAHAALDQPLPTTLKKQEEKEILKSQLDSLLGLYHLLDWFAVDESNEVDPEFSARLTGIKLEMEPSLSFYNKARNYATKKPYSVEKFKLNFQMPTLASGWDVNKEKNNGAILFVKNGLYYLGIMPKQKGRYKALSFEPTEKTSEGFDKMYYDYFPDAAKMIPKCSTQLKAVTAHFQTHTTPILLSNNFIEPLEITKEIYDLNNPEKEPKKFQTAYAKKTGDQKGYREALCKWIDFTRDFLSKYTKTTSIDLSSLRPSSQYKDLGEYYAELNPLLYHISFQRIAEKEIMDAVETGKLYLFQIYNKDFAKGHHGKPNLHTLYWTGLFSPENLAKTSIKLNGQAELFYRPKSRMKRMAHRLGEKMLNKKLKDQKTPIPDTLYQELYDYVNHRLSHDLSDEARALLPNVITKEVSHEIIKDRRFTSDKFFFHVPITLNYQAANSPSKFNQRVNAYLKEHPETPIIGIDRGERNLIYITVIDSTGKILEQRSLNTIQQFDYQKKLDNREKERVAARQAWSVVGTIKDLKQGYLSQVIHEIVDLMIHYQAVVVLENLNFGFKSKRTGIAEKAVYQQFEKMLIDKLNCLVLKDYPAEKVGGVLNPYQLTDQFTSFAKMGTQSGFLFYVPAPYTSKIDPLTGFVDPFVWKTIKNHESRKHFLEGFDFLHYDVKTGDFILHFKMNRNLSFQRGLPGFMPAWDIVFEKNETQFDAKGTPFIAGKRIVPVIENHRFTGRYRDLYPANELIALLEEKGIVFRDGSNILPKLLENDDSHAIDTMVALIRSVLQMRNSNAATGEDYINSPVRDLNGVCFDSRFQNPEWPMDADANGAYHIALKGQLLLNHLKESKDLKLQNGISNQDWLAYIQELRN

SEQ ID NO: 49 - protein, 1129 aa, Artificial Sequence
  Amino acid sequence WT AaCas12b
MAVKSMKVKLRLDNMPEIRAGLWKLHTEVNAGVRYYTEWLSLLRQENLYRRSPNGDGEQECYKTAEECKAELLERLRARQVENGHCGPAGSDDELLQLARQLYELLVPQAIGAKGDAQQIARKFLSPLADKDAVGGLGIAKAGNKPRWVRMREAGEPGWEEEKAKAEARKSTDRTADVLRALADFGLKPLMRVYTDSDMSSVQWKPLRKGQAVRTWDRDMFQQAIERMMSWESWNQRVGEAYAKLVEQKSRFEQKNFVGQEHLVQLVNQLQQDMKEASHGLESKEQTAHYLTGRALRGSDKVFEKWEKLDPDAPFDLYDTEIKNVQRRNTRRFGSHDLFAKLAEPKYQALWREDASFLTRYAVYNSIVRKLNHAKMFATFTLPDATAHPIWTRFDKLGGNLHQYTFLFNEFGEGRHAIRFQKLLTVEDGVAKEVDDVTVPISMSAQLDDLLPRDPHELVALYFQDYGAEQHLAGEFGGAKIQYRRDQLNHLHARRGARDVYLNLSVRVQSQSEARGERRPPYAAVFRLVGDNHRAFVHFDKLSDYLAEHPDDGKLGSEGLLSGLRVMSVDLGLRTSASISVFRVARKDELKPNSEGRVPFCFPIEGNENLVAVHERSQLLKLPGETESKDLRAIREERQRTLRQLRTQLAYLRLLVRCGSEDVGRRERSWAKLIEQPMDANQMTPDWREAFEDELQKLKSLYGICGDREWTEAVYESVRRVWRHMGKQVRDWRKDVRSGERPKIRGYQKDVVGGNSIEQIEYLERQYKFLKSWSFFGKVSGQVIRAEKGSRFAITLREHIDHAKEDRLKKLADRIIMEALGYVYALDDERGKGKWVAKYPPCQLILLEELSEYQFNNDRPPSENNQLMQWSHRGVFQELLNQAQVHDLLVGTMYAAFSSRFDARTGAPGIRCRRVPARCAREQNPEPFPWWLNKFVAEHKLDGCPLRADDLIPTGEGEFFVSPFSAEEGDFHQIHADLNAAQNLQRRLWSDFDISQIRLRCDWGEVDGEPVLIPRTTGKRTADSYGNKVFYTKTGVTYYERERGKKRRKVFAQEELSEEEAELLVEADEAREKSVVLMRDPSGIINRGDWTRQKEFWSMVNQRIEGYLVKQIRSRVRLQESACENTGDI

SEQ ID NO: 50 - protein, 1258 aa, Artificial Sequence
  Amino acid sequence WT Cas12d1
MNEKKTATQRRNARRRRGERARTKSQELRGYRLHDARIEFSGGLGSMRTVKVELLNPDSSREDPQRGQGLQGKVAKAVFDDYRALYGPMNIEDYLSDPDCPSFLGLWVKAVCLGVIMSRKTATDFGELRGGSKSGQAFDSIPEHLRRQLIKLKWLDWYDKGIRKSSSKASRLKSLTDVFANPKQPDQGVMAAWEQGEKLAESSRDIAALGRREFKDKLFAIPPPTSSVVLDDDVKATKVSRDWQWAVDPQFKLPSTDLDITRALEEVDRQWFERLGNNRGMVQQFFAIGDNGNHLNNGLFGHFFASIRSANLADIVAEMGTAFGFSAEERDIVRQRLETLHEYAQGLPEKPVLASRWAEYRTDMTAKLGSWYSNRTSKGAASITQVWGTINTETGEVKDDGLVRTLENIQSDLPDSCSIKEGILQETLDFIGDRRSSTDRAFTDELELYLATLRSDLNTWCQEQSALWEEKQRQVATPASDEKSKKADNPWAGKGSKTDKWLGALHTRIQSSPLFWGVDKLELWKTLANLKQAIRDEIDKLNEQVEVFGRSAYDEPVGKDADSGEGDRRVDQLSYLSARLGDQAHEEVRQRLDAIALALGVKFSERDDLHRFFVSSRARRRAALLAMPNTITVGKLRELADLTPLWERIKKKPEEPRLLADTVALSKVVNSACASRANPSDQIELTTIHSRLDGYSKNIGHTEFISRATVQSTNGAQNTVALDSLVSPRLFYYNFPNIVESAEPHVSHLEVATRGNLGSFEEFAAKEHRTFDRENPQKDSRNRIDSVNPLAVASSRYQIQFFTWWAGLHRSKETALEVGGSFTIAERQVRLDWSQEKPQAVVSEELRVFVSQPFTIVPDDKKRPATSGTRYIGVDIGEYGLAWSCWEFAPGYWNGSVVNPSKVTCLDYGFLAEPGQRRIVERVKKLRESQATKTFTSPDTYIARLRENVVATYQAQLEALMMAYNAQLVFESEISAFETGGNRVKKIYDAIKRSSVFGRSDAEATDNNQHWGKNGNRSSVKDPDKLRLNEAGQVAARVPWAEPVSAWMTSQTCSACGRVYVRAYRGKNSNEPDSGATGEVRYFDNKQQKILTKTIGADTVWVTDQERKEFERGVYNAMRPNAFMPDGRWTAAGEILEAALKSRGTLDGGRGFAGLHLTSKAQVHEYIEGTGKSHRDAHGNSAIFICPYTDCGHIADADLQASYNIALRGFAYAIVRKKHPELFAGSGSSTDGDEGGGKKPQQKQAFIDEIVRAAGRAS

SEQ ID NO: 51 - DNA, 3921 bp, Artificial Sequence
  Humanised nucleotide sequence WT AsCas12a
atgacacagttcgagggctttaccaacctgtatcaggtgagcaagacactgcggtttgagctgatcccacagggcaagaccctgaagcacatccaggagcagggcttcatcgaggaggacaaggcccgcaatgatcactacaaggagctgaagcccatcatcgatcggatctacaagacctatgccgaccagtgcctgcagctggtgcagctggattgggagaacctgagcgccgccatcgactcctatagaaaggagaaaaccgaggagacaaggaacgccctgatcgaggagcaggccacatatcgcaatgccatccacgactacttcatcggccggacagacaacctgaccgatgccatcaataagagacacgccgagatctacaagggcctgttcaaggccgagctgtttaatggcaaggtgctgaagcagctgggcaccgtgaccacaaccgagcacgagaacgccctgctgcggagcttcgacaagtttacaacctacttctccggcttttatgagaacaggaagaacgtgttcagcgccgaggatatcagcacagccatcccacaccgcatcgtgcaggacaacttccccaagtttaaggagaattgtcacatcttcacacgcctgatcaccgccgtgcccagcctgcgggagcactttgagaacgtgaagaaggccatcggcatcttcgtgagcacctccatcgaggaggtgttttccttccctttttataaccagctgctgacacagacccagatcgacctgtataaccagctgctgggaggaatctctcgggaggcaggcaccgagaagatcaagggcctgaacgaggtgctgaatctggccatccagaagaatgatgagacagcccacatcatcgcctccctgccacacagattcatccccctgtttaagcagatcctgtccgataggaacaccctgtctttcatcctggaggagtttaagagcgacgaggaagtgatccagtccttctgcaagtacaagacactgctgagaaacgagaacgtgctggagacagccgaggccctgtttaacgagctgaacagcatcgacctgacacacatcttcatcagccacaagaagctggagacaatcagcagcgccctgtgcgaccactgggatacactgaggaatgccctgtatgagcggagaatctccgagctgacaggcaagatcaccaagtctgccaaggagaaggtgcagcgcagcctgaagcacgaggatatcaacctgcaggagatcatctctgccgcaggcaaggagctgagcgaggccttcaagcagaaaaccagcgagatcctgtcccacgcacacgccgccctggatcagccactgcctacaaccctgaagaagcaggaggagaaggagatcctgaagtctcagctggacagcctgctgggcctgtaccacctgctggactggtttgccgtggatgagtccaacgaggtggaccccgagttctctgcccggctgaccggcatcaagctggagatggagccttctctgagcttctacaacaaggccagaaattatgccaccaagaagccctactccgtggagaagttcaagctgaactttcagatgcctacactggcctctggctgggacgtgaataaggagaagaacaatggcgccatcctgtttgtgaagaacggcctgtactatctgggcatcatgccaaagcagaagggcaggtataaggccctgagcttcgagcccacagagaaaaccagcgagggctttgataagatgtactatgactacttccctgatgccgccaagatgatcccaaagtgcagcacccagctgaaggccgtgacagcccactttcagacccacacaacccccatcctgctgtccaacaatttcatcgagcctctggagatcacaaaggagatctacgacctgaacaatcctgagaaggagccaaagaagtttcagacagcctacgccaagaaaaccggcgaccagaagggctacagagaggccctgtgcaagtggatcgacttcacaagggattttctgtccaagtataccaagacaacctctatcgatctgtctagcctgcggccatcctctcagtataaggacctgggcgagtactatgccgagctgaatcccctgctgtaccacatcagcttccagagaatcgccgagaaggagatcatggatgccgtggagacaggcaagctgtacctgttccagatctataacaaggactttgccaagggccaccacggcaagcctaatctgcacacactgtattggaccggcctgttttctccagagaacctggccaagacaagcatcaagctgaatggccaggccgagctgttctaccgccctaagtccaggatgaagaggatggcacaccggctgggagagaagatgctgaacaagaagctgaaggatcagaaaaccccaatccccgacaccctgtaccaggagctgtacgactatgtgaatcacagactgtcccacgacctgtctgatgaggccagggccctgctgcccaacgtgatcaccaaggaggtgtctcacgagatcatcaaggataggcgctttaccagcgacaagttctttttccacgtgcctatcacactgaactatcaggccgccaattccccatctaagttcaaccagagggtgaatgcctacctgaaggagcaccccgagacacctatcatcggcatcgatcggggcgagagaaacctgatctatatcacagtgatcgactccaccggcaagatcctggagcagcggagcctgaacaccatccagcagtttgattaccagaagaagctggacaacagggagaaggagagggtggcagcaaggcaggcctggtctgtggtgggcacaatcaaggatctgaagcagggctatctgagccaggtcatccacgagatcgtggacctgatgatccactaccaggccgtggtggtgctggagaacctgaatttcggctttaagagcaagaggaccggcatcgccgagaaggccgtgtaccagcagttcgagaagatgctgatcgataagctgaattgcctggtgctgaaggactatccagcagagaaagtgggaggcgtgctgaacccataccagctgacagaccagttcacctcctttgccaagatgggcacccagtctggcttcctgttttacgtgcctgccccatatacatctaagatcgatcccctgaccggcttcgtggaccccttcgtgtggaaaaccatcaagaatcacgagagccgcaagcacttcctggagggcttcgactttctgcactacgacgtgaaaaccggcgacttcatcctgcactttaagatgaacagaaatctgtccttccagaggggcctgcccggctttatgcctgcatgggatatcgtgttcgagaagaacgagacacagtttgacgccaagggcacccctttcatcgccggcaagagaatcgtgccagtgatcgagaatcacagattcaccggcagataccgggacctgtatcctgccaacgagctgatcgccctgctggaggagaagggcatcgtgttcagggatggctccaacatcctgccaaagctgctggagaatgacgattctcacgccatcgacaccatggtggccctgatccgcagcgtgctgcagatgcggaactccaatgccgccacaggcgaggactatatcaacagccccgtgcgcgatctgaatggcgtgtgcttcgactcccggtttcagaacccagagtggcccatggacgccgatgccaatggcgcctaccacatcgccctgaagggccagctgctgctgaatcacctgaaggagagcaaggatctgaagctgcagaacggcatctccaatcaggactggctggcctacatccaggagctgcgcaac

SEQ ID NO: 52 - DNA, 3387 bp, Artificial Sequence
  Humanised nucleotide sequence WT AaCas12b
atggccgtgaagagcatgaaggtgaagctgcgcctggacaacatgcccgagatccgcgccggcctgtggaagctgcacaccgaggtgaacgccggcgtgcgctactacaccgagtggctgagcctgctgcgccaggagaacctgtaccgccgcagccccaacggcgacggcgagcaggagtgctacaagaccgccgaggagtgcaaggccgagctgctggagcgcctgcgcgcccgccaggtggagaacggccactgcggccccgccggcagcgacgacgagctgctgcagctggcccgccagctgtacgagctgctggtgccccaggccatcggcgccaagggcgacgcccagcagatcgcccgcaagttcctgagccccctggccgacaaggacgccgtgggcggcctgggcatcgccaaggccggcaacaagccccgctgggtgcgcatgcgcgaggccggcgagcccggctgggaggaggagaaggccaaggccgaggcccgcaagagcaccgaccgcaccgccgacgtgctgcgcgccctggccgacttcggcctgaagcccctgatgcgcgtgtacaccgacagcgacatgagcagcgtgcagtggaagcccctgcgcaagggccaggccgtgcgcacctgggaccgcgacatgttccagcaggccatcgagcgcatgatgagctgggagagctggaaccagcgcgtgggcgaggcctacgccaagctggtggagcagaagagccgcttcgagcagaagaacttcgtgggccaggagcacctggtgcagctggtgaaccagctgcagcaggacatgaaggaggccagccacggcctggagagcaaggagcagaccgcccactacctgaccggccgcgccctgcgcggcagcgacaaggtgttcgagaagtgggagaagctggaccccgacgcccccttcgacctgtacgacaccgagatcaagaacgtgcagcgccgcaacacccgccgcttcggcagccacgacctgttcgccaagctggccgagcccaagtaccaggccctgtggcgcgaggacgccagcttcctgacccgctacgccgtgtacaacagcatcgtgcgcaagctgaaccacgccaagatgttcgccaccttcaccctgcccgacgccaccgcccaccccatctggacccgcttcgacaagctgggcggcaacctgcaccagtacaccttcctgttcaacgagttcggcgagggccgccacgccatccgcttccagaagctgctgaccgtggaggacggcgtggccaaggaggtggacgacgtgaccgtgcccatcagcatgagcgcccagctggacgacctgctgccccgcgacccccacgagctggtggccctgtacttccaggactacggcgccgagcagcacctggccggcgagttcggcggcgccaagatccagtaccgccgcgaccagctgaaccacctgcacgcccgccgcggcgcccgcgacgtgtacctgaacctgagcgtgcgcgtgcagagccagagcgaggcccgcggcgagcgccgccccccctacgccgccgtgttccgcctggtgggcgacaaccaccgcgccttcgtgcacttcgacaagctgagcgactacctggccgagcaccccgacgacggcaagctgggcagcgagggcctgctgagcggcctgcgcgtgatgagcgtggacctgggcctgcgcaccagcgccagcatcagcgtgttccgcgtggcccgcaaggacgagctgaagcccaacagcgagggccgcgtgcccttctgcttccccatcgagggcaacgagaacctggtggccgtgcacgagcgcagccagctgctgaagctgcccggcgagaccgagagcaaggacctgcgcgccatccgcgaggagcgccagcgcaccctgcgccagctgcgcacccagctggcctacctgcgcctgctggtgcgctgcggcagcgaggacgtgggccgccgcgagcgcagctgggccaagctgatcgagcagcccatggacgccaaccagatgacccccgactggcgcgaggccttcgaggacgagctgcagaagctgaagagcctgtacggcatctgcggcgaccgcgagtggaccgaggccgtgtacgagagcgtgcgccgcgtgtggcgccacatgggcaagcaggtgcgcgactggcgcaaggacgtgcgcagcggcgagcgccccaagatccgcggctaccagaaggacgtggtgggcggcaacagcatcgagcagatcgagtacctggagcgccagtacaagttcctgaagagctggagcttcttcggcaaggtgagcggccaggtgatccgcgccgagaagggcagccgcttcgccatcaccctgcgcgagcacatcgaccacgccaaggaggaccgcctgaagaagctggccgaccgcatcatcatggaggccctgggctacgtgtacgccctggacgacgagcgcggcaagggcaagtgggtggccaagtaccccccctgccagctgatcctgctggaggagctgagcgagtaccagttcaacaacgaccgcccccccagcgagaacaaccagctgatgcagtggagccaccgcggcgtgttccaggagctgctgaaccaggcccaggtgcacgacctgctggtgggcaccatgtacgccgccttcagcagccgcttcgacgcccgcaccggcgcccccggcatccgctgccgccgcgtgcccgcccgctgcgcccgcgagcagaaccccgagcccttcccctggtggctgaacaagttcgtggccgagcacaagctggacggctgccccctgcgcgccgacgacctgatccccaccggcgagggcgagttcttcgtgagccccttcagcgccgaggagggcgacttccaccagatccacgccgacctgaacgccgcccagaacctgcagcgccgcctgtggagcgacttcgacatcagccagatccgcctgcgctgcgactggggcgaggtggacggcgagcccgtgctgatcccccgcaccaccggcaagcgcaccgccgacagctacggcaacaaggtgttctacaccaagaccggcgtgacctactacgagcgcgagcgcggcaagaagcgccgcaaggtgttcgcccaggaggagctgagcgaggaggaggccgagctgctggtggaggccgacgaggcccgcgagaagagcgtggtgctgatgcgcgaccccagcggcatcatcaaccgcggcgactggacccgccagaaggagttctggagcatggtgaaccagcgcatcgagggctacctggtgaagcagatccgcagccgcgtgcgcctgcaggagagcgcctgcgagaacaccggcgacatc

SEQ ID NO: 53 - DNA, 3774 bp, Artificial Sequence
  Humanised nucleotide sequence WT Cas12d15
atgaacgaaaagaagaccgccacacagagaaggaacgcgcgcagaagaagaggagagagagccagaaccaagagccaggagttgagaggctaccggctgcacgacgccagaatcgagttcagcggcggactcggcagcatgagaacagtgaaggtggaactgctgaaccccgacagctccagagaggatccacagagaggccagggcctgcagggtaaagtggccaaggccgtgttcgacgactacagagccctgtacggccctatgaacatcgaggattatctgagcgaccctgactgcccttcttttctgggcctgtgggttaaggccgtttgtctgggcgtgatcatgagcagaaagaccgccaccgacttcggcgaattacgcggaggctctaagagcggacaggcgttcgatagcattcccgagcacctgagaagacaactgatcaaactgaagtggctggactggtacgacaagggcatccggaagtcctccagcaaggcctctcgtctgaagtccctgaccgacgtgttcgccaatcctaagcagcctgaccagggagttatggccgcgtgggagcagggcgagaagcttgctgaaagctccagagacattgcggccctgggaaggcgggaatttaaggacaagctgtttgctatccctccaccaacctcttccgtggtgttggatgacgacgtgaaggctaccaaggtgagccgcgattggcagtgggccgtggacccccagttcaagctgccgagcaccgacctggatatcaccagagccctggaggaagtggaccggcagtggttcgaacgcctgggcaataacagaggcatggtgcagcagttcttcgctatcggcgataacggcaaccacctgaacaacggcctgttcggccacttcttcgcctcgatcagaagtgccaacctggccgatatcgtggccgaaatgggcaccgcctttggttttagcgctgaggaaagagatatcgtgcggcagcggctggagaccctgcacgagtacgcccagggcctgcccgagaaacctgtcctggctagcagatgggccgagtacagaacagatatgacagccaagctgggcagttggtacagcaacagaacctccaagggcgccgcatctatcacacaggtgtggggcacaatcaacaccgagaccggagaggtgaaggatgatggactagtcagaaccctggaaaacatccagagcgatttgcctgacagctgtagcattaaagaaggcatcctgcaagagaccctggacttcatcggagatagacggagcagcacagacagagctttcacagacgaactggagctgtacctggctaccctacggagcgacctgaacacctggtgccaggagcagagcgccttgtgggaggaaaagcagcggcaggtcgctacgcctgcctctgatgagaaaagcaaaaaggccgacaatccatgggccggcaagggctccaaaacagataagtggctgggcgccctgcatacccggatccaaagcagccccctgttctggggcgtggacaagctggagctgtggaagaccctggccaacctgaagcaagccatcagagacgagatagacaagctgaacgagcaggtggaggtgttcgggagaagcgcctatgacgaacccgtaggcaaagatgcggactcaggagagggagatcggagagtggaccagctgagctacctgagtgccagactgggtgatcaggctcatgaagaggtcagacaacggctggacgccatcgccctggccctcggcgtgaagttctccgagcgggatgatcttcaccggtttttcgtgtctagcagagccagacggcgggctgccctgctggcgatgcccaataccatcacagtgggcaagctgcgggagctggctgacctgacaccactgtgggaacggatcaagaaaaagcctgaggagccaagactgctggccgatacagtggccctcagcaaggtggtgaacagcgcttgtgccagccgggctaatcctagcgaccagatcgagcttacaaccatccactctcggctcgacggctactccaagaacatcggacacacagagttcatcagcagagctacggtccagagcaccaacggagcccagaacaccgtcgccctggacagcctggtgagccccagactcttctactacaacttccccaatatcgtggaaagcgcagaaccccacgtgtcgcacctggaagtggccacaagaggcaatctggggtctttcgaagaattcgccgccaaggaacaccggaccttcgacagagaaaaccctcagaaagactccagaaaccggatcgatagcgttaaccctctggccgtggccagtagccggtaccagatccagttcttcacctggtgggccggcctgcacaggagcaaggagacagccctggaggtcggcggatcttttaccatcgccgaacggcaagtgcgtctggattggtcccaggagaaaccccaggccgtggtgtctgaagaactgagggtgttcgtgtctcaaccttttaccatcgtgcctgatgacaagaagcggcctgctaccagcggcacccggtacatcggcgtggacatcggcgagtacggcctcgcctggagctgctgggaattcgcccctggctactggaatggttctgttgtgaatcccagcaaggtgacatgcctggactacggattcctggccgaaccaggccagagaagaatcgtggagagagtgaagaagctgagagagagccaggccaccaagacattcaccagccctgatacctacatcgctcgtctgagagagaatgtggtggctacataccaagcccagctggaagcgctgatgatggcctacaacgcccaactggtgttcgagtccgagatctctgcctttgaaacaggaggcaaccgggtcaagaaaatctacgacgcaattaaaaggtctagcgtgtttggccgcagcgacgctgaggccaccgacaataaccagcactggggcaagaacggcaacagaagctccgtgaaggaccccgacaagctgaggctgaatgaggccggccaggtggccgccagagtgccttgggccgagcctgtgtccgcatggatgaccagccaaacatgcagcgcctgcggccgggtgtacgtgagagcctaccgaggcaagaactctaacgaacctgatagcggcgctacaggcgaagtgagatatttcgacaacaagcagcagaagatcctgaccaagaccatcggcgccgacaccgtgtgggtgaccgatcaggagagaaaagagttcgagcggggcgtttataacgccatgcgccccaacgccttcatgcctgacggcagatggaccgccgctggcgagattctggaagccgccctcaaaagcagaggaaccctggacggcggcagaggcttcgctggactgcacctgacatctaaggcccaggtgcacgagtacatcgagggcacaggcaagagccaccgggacgcccacggcaactccgcaatcttcatctgcccttacaccgactgcggccatatcgccgacgccgacctgcaggccagctacaacatcgccctgagaggcttcgcatacgccatcgtacggaagaagcaccctgagctgttcgcaggatctggcagctctactgacggcgacgaggggggaggcaaaaagcctcagcagaagcaggcctttatcgacgagattgtcagagccgccggcagagcctcc

SEQ ID NO: 54 - DNA, 3921 bp, Artificial Sequence
  Humanised nucleotide sequence dCas12a
atgacacagttcgagggctttaccaacctgtatcaggtgagcaagacactgcggtttgagctgatcccacagggcaagaccctgaagcacatccaggagcagggcttcatcgaggaggacaaggcccgcaatgatcactacaaggagctgaagcccatcatcgatcggatctacaagacctatgccgaccagtgcctgcagctggtgcagctggattgggagaacctgagcgccgccatcgactcctatagaaaggagaaaaccgaggagacaaggaacgccctgatcgaggagcaggccacatatcgcaatgccatccacgactacttcatcggccggacagacaacctgaccgatgccatcaataagagacacgccgagatctacaagggcctgttcaaggccgagctgtttaatggcaaggtgctgaagcagctgggcaccgtgaccacaaccgagcacgagaacgccctgctgcggagcttcgacaagtttacaacctacttctccggcttttatgagaacaggaagaacgtgttcagcgccgaggatatcagcacagccatcccacaccgcatcgtgcaggacaacttccccaagtttaaggagaattgtcacatcttcacacgcctgatcaccgccgtgcccagcctgcgggagcactttgagaacgtgaagaaggccatcggcatcttcgtgagcacctccatcgaggaggtgttttccttccctttttataaccagctgctgacacagacccagatcgacctgtataaccagctgctgggaggaatctctcgggaggcaggcaccgagaagatcaagggcctgaacgaggtgctgaatctggccatccagaagaatgatgagacagcccacatcatcgcctccctgccacacagattcatccccctgtttaagcagatcctgtccgataggaacaccctgtctttcatcctggaggagtttaagagcgacgaggaagtgatccagtccttctgcaagtacaagacactgctgagaaacgagaacgtgctggagacagccgaggccctgtttaacgagctgaacagcatcgacctgacacacatcttcatcagccacaagaagctggagacaatcagcagcgccctgtgcgaccactgggatacactgaggaatgccctgtatgagcggagaatctccgagctgacaggcaagatcaccaagtctgccaaggagaaggtgcagcgcagcctgaagcacgaggatatcaacctgcaggagatcatctctgccgcaggcaaggagctgagcgaggccttcaagcagaaaaccagcgagatcctgtcccacgcacacgccgccctggatcagccactgcctacaaccctgaagaagcaggaggagaaggagatcctgaagtctcagctggacagcctgctgggcctgtaccacctgctggactggtttgccgtggatgagtccaacgaggtggaccccgagttctctgcccggctgaccggcatcaagctggagatggagccttctctgagcttctacaacaaggccagaaattatgccaccaagaagccctactccgtggagaagttcaagctgaactttcagatgcctacactggcctctggctgggacgtgaataaggagaagaacaatggcgccatcctgtttgtgaagaacggcctgtactatctgggcatcatgccaaagcagaagggcaggtataaggccctgagcttcgagcccacagagaaaaccagcgagggctttgataagatgtactatgactacttccctgatgccgccaagatgatcccaaagtgcagcacccagctgaaggccgtgacagcccactttcagacccacacaacccccatcctgctgtccaacaatttcatcgagcctctggagatcacaaaggagatctacgacctgaacaatcctgagaaggagccaaagaagtttcagacagcctacgccaagaaaaccggcgaccagaagggctacagagaggccctgtgcaagtggatcgacttcacaagggattttctgtccaagtataccaagacaacctctatcgatctgtctagcctgcggccatcctctcagtataaggacctgggcgagtactatgccgagctgaatcccctgctgtaccacatcagcttccagagaatcgccgagaaggagatcatggatgccgtggagacaggcaagctgtacctgttccagatctataacaaggactttgccaagggccaccacggcaagcctaatctgcacacactgtattggaccggcctgttttctccagagaacctggccaagacaagcatcaagctgaatggccaggccgagctgttctaccgccctaagtccaggatgaagaggatggcacaccggctgggagagaagatgctgaacaagaagctgaaggatcagaaaaccccaatccccgacaccctgtaccaggagctgtacgactatgtgaatcacagactgtcccacgacctgtctgatgaggccagggccctgctgcccaacgtgatcaccaaggaggtgtctcacgagatcatcaaggataggcgctttaccagcgacaagttctttttccacgtgcctatcacactgaactatcaggccgccaattccccatctaagttcaaccagagggtgaatgcctacctgaaggagcaccccgagacacctatcatcggcatcgcccggggcgagagaaacctgatctatatcacagtgatcgactccaccggcaagatcctggagcagcggagcctgaacaccatccagcagtttgattaccagaagaagctggacaacagggagaaggagagggtggcagcaaggcaggcctggtctgtggtgggcacaatcaaggatctgaagcagggctatctgagccaggtcatccacgagatcgtggacctgatgatccactaccaggccgtggtggtgctggagaacctgaatttcggctttaagagcaagaggaccggcatcgccgagaaggccgtgtaccagcagttcgagaagatgctgatcgataagctgaattgcctggtgctgaaggactatccagcagagaaagtgggaggcgtgctgaacccataccagctgacagaccagttcacctcctttgccaagatgggcacccagtctggcttcctgttttacgtgcctgccccatatacatctaagatcgatcccctgaccggcttcgtggaccccttcgtgtggaaaaccatcaagaatcacgagagccgcaagcacttcctggagggcttcgactttctgcactacgacgtgaaaaccggcgacttcatcctgcactttaagatgaacagaaatctgtccttccagaggggcctgcccggctttatgcctgcatgggatatcgtgttcgagaagaacgagacacagtttgacgccaagggcacccctttcatcgccggcaagagaatcgtgccagtgatcgagaatcacagattcaccggcagataccgggacctgtatcctgccaacgagctgatcgccctgctggaggagaagggcatcgtgttcagggatggctccaacatcctgccaaagctgctggagaatgacgattctcacgccatcgacaccatggtggccctgatccgcagcgtgctgcagatgcggaactccaatgccgccacaggcgaggactatatcaacagccccgtgcgcgatctgaatggcgtgtgcttcgactcccggtttcagaacccagagtggcccatggacgccgatgccaatggcgcctaccacatcgccctgaagggccagctgctgctgaatcacctgaaggagagcaaggatctgaagctgcagaacggcatctccaatcaggactggctggcctacatccaggagctgcgcaac

SEQ ID NO: 55 - DNA, 3387 bp, Artificial Sequence
  Humanised nucleotide sequence dCas12b
atggccgtgaagagcatgaaggtgaagctgcgcctggacaacatgcccgagatccgcgccggcctgtggaagctgcacaccgaggtgaacgccggcgtgcgctactacaccgagtggctgagcctgctgcgccaggagaacctgtaccgccgcagccccaacggcgacggcgagcaggagtgctacaagaccgccgaggagtgcaaggccgagctgctggagcgcctgcgcgcccgccaggtggagaacggccactgcggccccgccggcagcgacgacgagctgctgcagctggcccgccagctgtacgagctgctggtgccccaggccatcggcgccaagggcgacgcccagcagatcgcccgcaagttcctgagccccctggccgacaaggacgccgtgggcggcctgggcatcgccaaggccggcaacaagccccgctgggtgcgcatgcgcgaggccggcgagcccggctgggaggaggagaaggccaaggccgaggcccgcaagagcaccgaccgcaccgccgacgtgctgcgcgccctggccgacttcggcctgaagcccctgatgcgcgtgtacaccgacagcgacatgagcagcgtgcagtggaagcccctgcgcaagggccaggccgtgcgcacctgggaccgcgacatgttccagcaggccatcgagcgcatgatgagctgggagagctggaaccagcgcgtgggcgaggcctacgccaagctggtggagcagaagagccgcttcgagcagaagaacttcgtgggccaggagcacctggtgcagctggtgaaccagctgcagcaggacatgaaggaggccagccacggcctggagagcaaggagcagaccgcccactacctgaccggccgcgccctgcgcggcagcgacaaggtgttcgagaagtgggagaagctggaccccgacgcccccttcgacctgtacgacaccgagatcaagaacgtgcagcgccgcaacacccgccgcttcggcagccacgacctgttcgccaagctggccgagcccaagtaccaggccctgtggcgcgaggacgccagcttcctgacccgctacgccgtgtacaacagcatcgtgcgcaagctgaaccacgccaagatgttcgccaccttcaccctgcccgacgccaccgcccaccccatctggacccgcttcgacaagctgggcggcaacctgcaccagtacaccttcctgttcaacgagttcggcgagggccgccacgccatccgcttccagaagctgctgaccgtggaggacggcgtggccaaggaggtggacgacgtgaccgtgcccatcagcatgagcgcccagctggacgacctgctgccccgcgacccccacgagctggtggccctgtacttccaggactacggcgccgagcagcacctggccggcgagttcggcggcgccaagatccagtaccgccgcgaccagctgaaccacctgcacgcccgccgcggcgcccgcgacgtgtacctgaacctgagcgtgcgcgtgcagagccagagcgaggcccgcggcgagcgccgccccccctacgccgccgtgttccgcctggtgggcgacaaccaccgcgccttcgtgcacttcgacaagctgagcgactacctggccgagcaccccgacgacggcaagctgggcagcgagggcctgctgagcggcctgcgcgtgatgagcgtggccctgggcctgcgcaccagcgccagcatcagcgtgttccgcgtggcccgcaaggacgagctgaagcccaacagcgagggccgcgtgcccttctgcttccccatcgagggcaacgagaacctggtggccgtgcacgagcgcagccagctgctgaagctgcccggcgagaccgagagcaaggacctgcgcgccatccgcgaggagcgccagcgcaccctgcgccagctgcgcacccagctggcctacctgcgcctgctggtgcgctgcggcagcgaggacgtgggccgccgcgagcgcagctgggccaagctgatcgagcagcccatggacgccaaccagatgacccccgactggcgcgaggccttcgaggacgagctgcagaagctgaagagcctgtacggcatctgcggcgaccgcgagtggaccgaggccgtgtacgagagcgtgcgccgcgtgtggcgccacatgggcaagcaggtgcgcgactggcgcaaggacgtgcgcagcggcgagcgccccaagatccgcggctaccagaaggacgtggtgggcggcaacagcatcgagcagatcgagtacctggagcgccagtacaagttcctgaagagctggagcttcttcggcaaggtgagcggccaggtgatccgcgccgagaagggcagccgcttcgccatcaccctgcgcgagcacatcgaccacgccaaggaggaccgcctgaagaagctggccgaccgcatcatcatggaggccctgggctacgtgtacgccctggacgacgagcgcggcaagggcaagtgggtggccaagtaccccccctgccagctgatcctgctggaggagctgagcgagtaccagttcaacaacgaccgcccccccagcgagaacaaccagctgatgcagtggagccaccgcggcgtgttccaggagctgctgaaccaggcccaggtgcacgacctgctggtgggcaccatgtacgccgccttcagcagccgcttcgacgcccgcaccggcgcccccggcatccgctgccgccgcgtgcccgcccgctgcgcccgcgagcagaaccccgagcccttcccctggtggctgaacaagttcgtggccgagcacaagctggacggctgccccctgcgcgccgacgacctgatccccaccggcgagggcgagttcttcgtgagccccttcagcgccgaggagggcgacttccaccagatccacgccgacctgaacgccgcccagaacctgcagcgccgcctgtggagcgacttcgacatcagccagatccgcctgcgctgcgactggggcgaggtggacggcgagcccgtgctgatcccccgcaccaccggcaagcgcaccgccgacagctacggcaacaaggtgttctacaccaagaccggcgtgacctactacgagcgcgagcgcggcaagaagcgccgcaaggtgttcgcccaggaggagctgagcgaggaggaggccgagctgctggtggaggccgacgaggcccgcgagaagagcgtggtgctgatgcgcgaccccagcggcatcatcaaccgcggcgactggacccgccagaaggagttctggagcatggtgaaccagcgcatcgagggctacctggtgaagcagatccgcagccgcgtgcgcctgcaggagagcgcctgcgagaacaccggcgacatc

SEQ ID NO: 56 - DNA, 3774 bp, Artificial Sequence
  Humanised nucleotide sequence dCas12d
atgaacgaaaagaagaccgccacacagagaaggaacgcgcgcagaagaagaggagagagagccagaaccaagagccaggagttgagaggctaccggctgcacgacgccagaatcgagttcagcggcggactcggcagcatgagaacagtgaaggtggaactgctgaaccccgacagctccagagaggatccacagagaggccagggcctgcagggtaaagtggccaaggccgtgttcgacgactacagagccctgtacggccctatgaacatcgaggattatctgagcgaccctgactgcccttcttttctgggcctgtgggttaaggccgtttgtctgggcgtgatcatgagcagaaagaccgccaccgacttcggcgaattacgcggaggctctaagagcggacaggcgttcgatagcattcccgagcacctgagaagacaactgatcaaactgaagtggctggactggtacgacaagggcatccggaagtcctccagcaaggcctctcgtctgaagtccctgaccgacgtgttcgccaatcctaagcagcctgaccagggagttatggccgcgtgggagcagggcgagaagcttgctgaaagctccagagacattgcggccctgggaaggcgggaatttaaggacaagctgtttgctatccctccaccaacctcttccgtggtgttggatgacgacgtgaaggctaccaaggtgagccgcgattggcagtgggccgtggacccccagttcaagctgccgagcaccgacctggatatcaccagagccctggaggaagtggaccggcagtggttcgaacgcctgggcaataacagaggcatggtgcagcagttcttcgctatcggcgataacggcaaccacctgaacaacggcctgttcggccacttcttcgcctcgatcagaagtgccaacctggccgatatcgtggccgaaatgggcaccgcctttggttttagcgctgaggaaagagatatcgtgcggcagcggctggagaccctgcacgagtacgcccagggcctgcccgagaaacctgtcctggctagcagatgggccgagtacagaacagatatgacagccaagctgggcagttggtacagcaacagaacctccaagggcgccgcatctatcacacaggtgtggggcacaatcaacaccgagaccggagaggtgaaggatgatggactagtcagaaccctggaaaacatccagagcgatttgcctgacagctgtagcattaaagaaggcatcctgcaagagaccctggacttcatcggagatagacggagcagcacagacagagctttcacagacgaactggagctgtacctggctaccctacggagcgacctgaacacctggtgccaggagcagagcgccttgtgggaggaaaagcagcggcaggtcgctacgcctgcctctgatgagaaaagcaaaaaggccgacaatccatgggccggcaagggctccaaaacagataagtggctgggcgccctgcatacccggatccaaagcagccccctgttctggggcgtggacaagctggagctgtggaagaccctggccaacctgaagcaagccatcagagacgagatagacaagctgaacgagcaggtggaggtgttcgggagaagcgcctatgacgaacccgtaggcaaagatgcggactcaggagagggagatcggagagtggaccagctgagctacctgagtgccagactgggtgatcaggctcatgaagaggtcagacaacggctggacgccatcgccctggccctcggcgtgaagttctccgagcgggatgatcttcaccggtttttcgtgtctagcagagccagacggcgggctgccctgctggcgatgcccaataccatcacagtgggcaagctgcgggagctggctgacctgacaccactgtgggaacggatcaagaaaaagcctgaggagccaagactgctggccgatacagtggccctcagcaaggtggtgaacagcgcttgtgccagccgggctaatcctagcgaccagatcgagcttacaaccatccactctcggctcgacggctactccaagaacatcggacacacagagttcatcagcagagctacggtccagagcaccaacggagcccagaacaccgtcgccctggacagcctggtgagccccagactcttctactacaacttccccaatatcgtggaaagcgcagaaccccacgtgtcgcacctggaagtggccacaagaggcaatctggggtctttcgaagaattcgccgccaaggaacaccggaccttcgacagagaaaaccctcagaaagactccagaaaccggatcgatagcgttaaccctctggccgtggccagtagccggtaccagatccagttcttcacctggtgggccggcctgcacaggagcaaggagacagccctggaggtcggcggatcttttaccatcgccgaacggcaagtgcgtctggattggtcccaggagaaaccccaggccgtggtgtctgaagaactgagggtgttcgtgtctcaaccttttaccatcgtgcctgatgacaagaagcggcctgctaccagcggcacccggtacatcggcgtggccatcggcgagtacggcctcgcctggagctgctgggaattcgcccctggctactggaatggttctgttgtgaatcccagcaaggtgacatgcctggactacggattcctggccgaaccaggccagagaagaatcgtggagagagtgaagaagctgagagagagccaggccaccaagacattcaccagccctgatacctacatcgctcgtctgagagagaatgtggtggctacataccaagcccagctggaagcgctgatgatggcctacaacgcccaactggtgttcgcctccgagatctctgcctttgaaacaggaggcaaccgggtcaagaaaatctacgacgcaattaaaaggtctagcgtgtttggccgcagcgacgctgaggccaccgacaataaccagcactggggcaagaacggcaacagaagctccgtgaaggaccccgacaagctgaggctgaatgaggccggccaggtggccgccagagtgccttgggccgagcctgtgtccgcatggatgaccagccaaacatgcagcgcctgcggccgggtgtacgtgagagcctaccgaggcaagaactctaacgaacctgatagcggcgctacaggcgaagtgagatatttcgacaacaagcagcagaagatcctgaccaagaccatcggcgccgacaccgtgtgggtgaccgatcaggagagaaaagagttcgagcggggcgtttataacgccatgcgccccaacgccttcatgcctgacggcagatggaccgccgctggcgagattctggaagccgccctcaaaagcagaggaaccctggacggcggcagaggcttcgctggactgcacctgacatctaaggcccaggtgcacgagtacatcgagggcacaggcaagagccaccgggacgcccacggcaactccgcaatcttcatctgcccttacaccgactgcggccatatcgccgacgccgccctgcaggccagctacaacatcgccctgagaggcttcgcatacgccatcgtacggaagaagcaccctgagctgttcgcaggatctggcagctctactgacggcgacgaggggggaggcaaaaagcctcagcagaagcaggcctttatcgacgagattgtcagagccgccggcagagcctcc

SEQ ID NO: 57 - protein, 1307 aa, Artificial Sequence
  Amino acid sequence dAsCas12a
MTQFEGFTNLYQVSKTLRFELIPQGKTLKHIQEQGFIEEDKARNDHYKELKPIIDRIYKTYADQCLQLVQLDWENLSAAIDSYRKEKTEETRNALIEEQATYRNAIHDYFIGRTDNLTDAINKRHAEIYKGLFKAELFNGKVLKQLGTVTTTEHENALLRSFDKFTTYFSGFYENRKNVFSAEDISTAIPHRIVQDNFPKFKENCHIFTRLITAVPSLREHFENVKKAIGIFVSTSIEEVFSFPFYNQLLTQTQIDLYNQLLGGISREAGTEKIKGLNEVLNLAIQKNDETAHIIASLPHRFIPLFKQILSDRNTLSFILEEFKSDEEVIQSFCKYKTLLRNENVLETAEALFNELNSIDLTHIFISHKKLETISSALCDHWDTLRNALYERRISELTGKITKSAKEKVQRSLKHEDINLQEIISAAGKELSEAFKQKTSEILSHAHAALDQPLPTTLKKQEEKEILKSQLDSLLGLYHLLDWFAVDESNEVDPEFSARLTGIKLEMEPSLSFYNKARNYATKKPYSVEKFKLNFQMPTLASGWDVNKEKNNGAILFVKNGLYYLGIMPKQKGRYKALSFEPTEKTSEGFDKMYYDYFPDAAKMIPKCSTQLKAVTAHFQTHTTPILLSNNFIEPLEITKEIYDLNNPEKEPKKFQTAYAKKTGDQKGYREALCKWIDFTRDFLSKYTKTTSIDLSSLRPSSQYKDLGEYYAELNPLLYHISFQRIAEKEIMDAVETGKLYLFQIYNKDFAKGHHGKPNLHTLYWTGLFSPENLAKTSIKLNGQAELFYRPKSRMKRMAHRLGEKMLNKKLKDQKTPIPDTLYQELYDYVNHRLSHDLSDEARALLPNVITKEVSHEIIKDRRFTSDKFFFHVPITLNYQAANSPSKFNQRVNAYLKEHPETPIIGIARGERNLIYITVIDSTGKILEQRSLNTIQQFDYQKKLDNREKERVAARQAWSVVGTIKDLKQGYLSQVIHEIVDLMIHYQAVVVLENLNFGFKSKRTGIAEKAVYQQFEKMLIDKLNCLVLKDYPAEKVGGVLNPYQLTDQFTSFAKMGTQSGFLFYVPAPYTSKIDPLTGFVDPFVWKTIKNHESRKHFLEGFDFLHYDVKTGDFILHFKMNRNLSFQRGLPGFMPAWDIVFEKNETQFDAKGTPFIAGKRIVPVIENHRFTGRYRDLYPANELIALLEEKGIVFRDGSNILPKLLENDDSHAIDTMVALIRSVLQMRNSNAATGEDYINSPVRDLNGVCFDSRFQNPEWPMDADANGAYHIALKGQLLLNHLKESKDLKLQNGISNQDWLAYIQELRN

SEQ ID NO: 58 - protein, 1129 aa, Artificial Sequence
  Amino acid sequence dAaCas12b
MAVKSMKVKLRLDNMPEIRAGLWKLHTEVNAGVRYYTEWLSLLRQENLYRRSPNGDGEQECYKTAEECKAELLERLRARQVENGHCGPAGSDDELLQLARQLYELLVPQAIGAKGDAQQIARKFLSPLADKDAVGGLGIAKAGNKPRWVRMREAGEPGWEEEKAKAEARKSTDRTADVLRALADFGLKPLMRVYTDSDMSSVQWKPLRKGQAVRTWDRDMFQQAIERMMSWESWNQRVGEAYAKLVEQKSRFEQKNFVGQEHLVQLVNQLQQDMKEASHGLESKEQTAHYLTGRALRGSDKVFEKWEKLDPDAPFDLYDTEIKNVQRRNTRRFGSHDLFAKLAEPKYQALWREDASFLTRYAVYNSIVRKLNHAKMFATFTLPDATAHPIWTRFDKLGGNLHQYTFLFNEFGEGRHAIRFQKLLTVEDGVAKEVDDVTVPISMSAQLDDLLPRDPHELVALYFQDYGAEQHLAGEFGGAKIQYRRDQLNHLHARRGARDVYLNLSVRVQSQSEARGERRPPYAAVFRLVGDNHRAFVHFDKLSDYLAEHPDDGKLGSEGLLSGLRVMSVALGLRTSASISVFRVARKDELKPNSEGRVPFCFPIEGNENLVAVHERSQLLKLPGETESKDLRAIREERQRTLRQLRTQLAYLRLLVRCGSEDVGRRERSWAKLIEQPMDANQMTPDWREAFEDELQKLKSLYGICGDREWTEAVYESVRRVWRHMGKQVRDWRKDVRSGERPKIRGYQKDVVGGNSIEQIEYLERQYKFLKSWSFFGKVSGQVIRAEKGSRFAITLREHIDHAKEDRLKKLADRIIMEALGYVYALDDERGKGKWVAKYPPCQLILLEELSEYQFNNDRPPSENNQLMQWSHRGVFQELLNQAQVHDLLVGTMYAAFSSRFDARTGAPGIRCRRVPARCAREQNPEPFPWWLNKFVAEHKLDGCPLRADDLIPTGEGEFFVSPFSAEEGDFHQIHADLNAAQNLQRRLWSDFDISQIRLRCDWGEVDGEPVLIPRTTGKRTADSYGNKVFYTKTGVTYYERERGKKRRKVFAQEELSEEEAELLVEADEAREKSVVLMRDPSGIINRGDWTRQKEFWSMVNQRIEGYLVKQIRSRVRLQESACENTGDI

SEQ ID NO: 59 - protein, 1258 aa, Artificial Sequence
  Amino acid sequence dCas12d15
MNEKKTATQRRNARRRRGERARTKSQELRGYRLHDARIEFSGGLGSMRTVKVELLNPDSSREDPQRGQGLQGKVAKAVFDDYRALYGPMNIEDYLSDPDCPSFLGLWVKAVCLGVIMSRKTATDFGELRGGSKSGQAFDSIPEHLRRQLIKLKWLDWYDKGIRKSSSKASRLKSLTDVFANPKQPDQGVMAAWEQGEKLAESSRDIAALGRREFKDKLFAIPPPTSSVVLDDDVKATKVSRDWQWAVDPQFKLPSTDLDITRALEEVDRQWFERLGNNRGMVQQFFAIGDNGNHLNNGLFGHFFASIRSANLADIVAEMGTAFGFSAEERDIVRQRLETLHEYAQGLPEKPVLASRWAEYRTDMTAKLGSWYSNRTSKGAASITQVWGTINTETGEVKDDGLVRTLENIQSDLPDSCSIKEGILQETLDFIGDRRSSTDRAFTDELELYLATLRSDLNTWCQEQSALWEEKQRQVATPASDEKSKKADNPWAGKGSKTDKWLGALHTRIQSSPLFWGVDKLELWKTLANLKQAIRDEIDKLNEQVEVFGRSAYDEPVGKDADSGEGDRRVDQLSYLSARLGDQAHEEVRQRLDAIALALGVKFSERDDLHRFFVSSRARRRAALLAMPNTITVGKLRELADLTPLWERIKKKPEEPRLLADTVALSKVVNSACASRANPSDQIELTTIHSRLDGYSKNIGHTEFISRATVQSTNGAQNTVALDSLVSPRLFYYNFPNIVESAEPHVSHLEVATRGNLGSFEEFAAKEHRTFDRENPQKDSRNRIDSVNPLAVASSRYQIQFFTWWAGLHRSKETALEVGGSFTIAERQVRLDWSQEKPQAVVSEELRVFVSQPFTIVPDDKKRPATSGTRYIGVAIGEYGLAWSCWEFAPGYWNGSVVNPSKVTCLDYGFLAEPGQRRIVERVKKLRESQATKTFTSPDTYIARLRENVVATYQAQLEALMMAYNAQLVFASEISAFETGGNRVKKIYDAIKRSSVFGRSDAEATDNNQHWGKNGNRSSVKDPDKLRLNEAGQVAARVPWAEPVSAWMTSQTCSACGRVYVRAYRGKNSNEPDSGATGEVRYFDNKQQKILTKTIGADTVWVTDQERKEFERGVYNAMRPNAFMPDGRWTAAGEILEAALKSRGTLDGGRGFAGLHLTSKAQVHEYIEGTGKSHRDAHGNSAIFICPYTDCGHIADAALQASYNIALRGFAYAIVRKKHPELFAGSGSSTDGDEGGGKKPQQKQAFIDEIVRAAGRAS

SEQ ID NO: 60 - protein, 84 aa, Artificial Sequence
  Bacillus phage PBS2 Uracil-DNA glycosylase inhibitor
MTNLSDIIEKETGKQLVIQESILMLPEEVEEVIGNKPESDILVHTAYDESTDENVMLLTSDAPEYKPWALVIQDSNGENKIKML

SEQ ID NO: 61 - RNA, 93 nt, Artificial Sequence
  Hybrid Type II crRNA:tracrRNA guide RNA sequence
guuuaagagcuaugcuggaaacagcauagcaaguuuaaauaaggcuaguccguuaucaacuugaaaaaguggcaccgagucggugcuuuuuuu

SEQ ID NO: 62 - DNA, 129 bp, Artificial Sequence
  RNA scaffold expression cassette (S. pyogenes), containing a 20-nucleotide programmable sequence, a CRISPR RNA motif, and an MS2 operator motif
  misc_feature (1)..(20): n is a, c, g, or t
nnnnnnnnnnnnnnnnnnnngttttagagctagaaatagcaagttaaaataaggctagtccgttatcaacttgaaaaagtggcaccgagtcggtgcgcgcacatgaggatcacccatgtgctttttttg

SEQ ID NO: 63 - DNA, 157 bp, Artificial Sequence
  RNA scaffold containing two MS2 loops (2xMS2)
gttttagagctagaaatagcaagttaaaataaggctagtccgttatcaacttgaaaaagtggcaccgagtcggtgcgggagcacatgaggatcacccatgtgccacgagcgacatgaggatcacccatgtcgctcgtgttccctttttttctccgct

SEQ ID NO: 64 - RNA, 957 nt, Artificial Sequence
  NLS-Anolis(P16A-E17A)-Apobec1-Linker-MCP RNA seq
auggcccccaagaagaagcggaaagugauggagccggaggcuuuucagcgcaacuuugacccucgggaauuugccgccuguacacuccucuuguaugagauccacugggacaauaacacaucuagaaauugguguacgaauaagccugggcuccacgcugaggagaauuucuugcagauauuuaaugagaaaauugacauuaaacaggauacgccgugcucuauaacaugguuccuuucuuggagccccuguuacccuuguagccaagcaauaauaaaauucuuggaggcacacccgaaugucagucuggagauuaaggcugcgcggcuguauaugcaucaaauagacuguaacaaggagggacucagaaaucugggccggaaucgagugucaauaaugaaccugccugauuauaggcauugcuggacuacguuuguugugccaaggggagcaaacgaagauuacuggccacaagacuuucugccugcgaucacaaauuacucccgagaacucgacuccauacugcaggaugagcugaagacaccccugggcgacaccacacacaccucuccaccuugcccagcaccagagcugcugggaggcccuauggccagcaacuucacacaguuugugcugguggauaauggaggaaccggcgacgugacaguggcaccaucuaacuuugccaauggcaucgccgaguggaucagcuccaacucucggagccaggccuauaaggugaccuguagcgugcggcagucuagcgcccagaauagaaaguauacaaucaagguggaggugccuaagggcgccuggagauccuaccugaacauggagcugaccaucccaaucuuugccacaaauucugauugcgagcugaucgugaaggccaugcagggccugcugaaggacggcaacccuaucccaagcgccaucgccgccaauagcggaaucuac

SEQ ID NO: 65 - RNA, 1137 nt, Artificial Sequence
  NLS-Rattus-Apobec1-Linker-MCP RNA seq
auggcccccaagaagaagcggaaaguguccucagagacugggccugucgccgucgauccaacccugcgccgccggauugaaccucacgaguuugaaguguucuuugacccccgggagcugagaaaggagacaugccugcuguacgagaucaacuggggaggcaggcacuccaucuggaggcacaccucucagaacacaaauaagcacguggaggugaacuucaucgagaaguuuaccacagagcgguacuucugccccaauaccagauguagcaucacaugguuucugagcugguccccuugcggagaguguagcagggccaucaccgaguuccuguccagauauccacacgugacacuguuuaucuacaucgccaggcuguaucaccacgcagacccaaggaauaggcagggccugcgcgaucugaucagcuccggcgugaccauccagaucaugacagagcaggaguccggcuacugcuggcggaacuucgugaauuauucuccuagcaacgaggcccacuggccuagguacccacaccugugggugcgccuguacgugcuggagcuguauugcaucauccugggccugcccccuugucugaauauccugcggagaaagcagccccagcugaccuucuuuacaaucgcccugcagucuugucacuaucagaggcugccaccccacauccugugggccacaggccugaaggagcugaagacaccccugggcgacaccacacacaccucuccaccuugcccagcaccagagcugcugggaggcccuauggccagcaacuucacacaguuugugcugguggauaauggaggaaccggcgacgugacaguggcaccaucuaacuuugccaauggcaucgccgaguggaucagcuccaacucucggagccaggccuauaaggugaccuguagcgugcggcagucuagcgcccagaauagaaaguauacaaucaagguggaggugccuaagggcgccuggagauccuaccugaacauggagcugaccaucccaaucuuugccacaaauucugauugcgagcugaucgugaaggccaugcagggccugcugaaggacggcaacccuaucccaagcgccaucgccgccaauagcggaaucuac

SEQ ID NO: 66 - RNA, 1047 nt, Artificial Sequence
  NLS-Homo-AID-L25-MCP RNA seq
auggcccccaagaagaagcggaaagugauggauagccugcugaugaaccggagaaaguuccuguaucaguuuaagaaugugcgcugggcaaagggcaggcgcgagaccuaccugugcuauguggugaagcggagagauuccgccacauccuucucucuggacuuuggcuaccugcggaacaagaauggcugccacguggagcugcuguuccugagauacaucucugacugggaucuggacccaggcagguguuaucgcgugaccugguucacaagcuggucccccugcuacgauugugcaaggcacguggcagacuuucugaggggaaacccaaaucugucccugcggaucuucaccgccagacuguauuuuugcgaggauaggaaggcagagccagagggacugaggcgccugcacagggccggcgugcagaucgccaucaugaccuucaaggacuacuuuuauuguuggaacaccuucguggagaaucacgagcggaccuucaaggccugggagggacugcacgagaacuccgugcggcugucuagacagcugcggagaauccugcugccucuguacgagguggacgaucugagggaugccuuccgcacccugggacuggagcugaagacaccccugggcgacaccacacacaccucuccaccuugcccagcaccagagcugcugggaggcccuauggccagcaacuucacacaguuugugcugguggauaauggaggaaccggcgacgugacaguggcaccaucuaacuuugccaauggcaucgccgaguggaucagcuccaacucucggagccaggccuauaaggugaccuguagcgugcggcagucuagcgcccagaauagaaaguauacaaucaagguggaggugccuaagggcgccuggagauccuaccugaacauggagcugaccaucccaaucuuugccacaaauucugauugcgagcugaucgugaaggccaugcagggccugcugaaggacggcaacccuaucccaagcgccaucgccgccaauagcggaaucuac

SEQ ID NO: 67 - RNA, 4746 nt, Artificial Sequence
  NLS-nCas9(D10A)-UGI-UGI-NLS RNA seq
augccaaagaagaagcggaaagucgacaagaaguacagcaucggccuggccaucggcaccaacucugugggcugggccgugaucaccgacgaguacaaggugcccagcaagaaauucaaggugcugggcaacaccgaccggcacagcaucaagaagaaccugaucggagcccugcuguucgacagcggcgaaacagccgaggccacccggcugaagagaaccgccagaagaagauacaccagacggaagaaccggaucugcuaucugcaagagaucuucagcaacgagauggccaagguggacgacagcuucuuccacagacuggaagaguccuuccugguggaagaggauaagaagcacgagcggcaccccaucuucggcaacaucguggacgagguggccuaccacgagaaguaccccaccaucuaccaccugagaaagaaacugguggacagcaccgacaaggccgaccugcggcugaucuaucuggcccuggcccacaugaucaaguuccggggccacuuccugaucgagggcgaccugaaccccgacaacagcgacguggacaagcuguucauccagcuggugcagaccuacaaccagcuguucgaggaaaaccccaucaacgccagcggcguggacgccaaggccauccugucugccagacugagcaagagcagacggcuggaaaaucugaucgcccagcugcccggcgagaagaagaauggccuguucggaaaccugauugcccugagccugggccugacccccaacuucaagagcaacuucgaccuggccgaggaugccaaacugcagcugagcaaggacaccuacgacgacgaccuggacaaccugcuggcccagaucggcgaccaguacgccgaccuguuucuggccgccaagaaccuguccgacgccauccugcugagcgacauccugagagugaacaccgagaucaccaaggccccccugagcgccucuaugaucaagagauacgacgagcaccaccaggaccugacccugcugaaagcucucgugcggcagcagcugccugagaaguacaaagagauuuucuucgaccagagcaagaacggcuacgccggcuacauugacggcggagccagccaggaagaguucuacaaguucaucaagcccauccuggaaaagauggacggcaccgaggaacugcucgugaagcugaacagagaggaccugcugcggaagcagcggaccuucgacaacggcagcaucccccaccagauccaccugggagagcugcacgccauucugcggcggcaggaagauuuuuacccauuccugaaggacaaccgggaaaagaucgagaagauccugaccuuccgcauccccuacuacgugggcccucuggccaggggaaacagcagauucgccuggaugaccagaaagagcgaggaaaccaucacccccuggaacuucgaggaagugguggacaagggcgcuuccgcccagagcuucaucgagcggaugaccaacuucgauaagaaccugcccaacgagaaggugcugcccaagcacagccugcuguacgaguacuucaccguguauaacgagcugaccaaagugaaauacgugaccgagggaaugagaaagcccgccuuccugagcggcgagcagaaaaaggccaucguggaccugcuguucaagaccaaccggaaagugaccgugaagcagcugaaagaggacuacuucaagaaaaucgagugcuucgacuccguggaaaucuccggcguggaagaucgguucaacgccucccugggcacauaccacgaucugcugaaaauuaucaaggacaaggacuuccuggacaaugaggaaaacgaggacauucuggaagauaucgugcugacccugacacuguuugaggacagagagaugaucgaggaacggcugaaaaccuaugcccaccuguucgacgacaaagugaugaagcagcugaagcggcggagauacaccggcuggggcaggcugagccggaagcugaucaacggcauccgggacaagcaguccggcaagacaauccuggauuuccugaaguccgacggcuucgccaacagaaacuucaugcagcugauccacgacgacagccugaccuuuaaagaggacauccagaaagcccagguguccggccagggcgauagccugcacgagcacauugccaaucuggccggcagccccgccauuaagaagggcauccugcagacagugaaggugguggacgagcucgugaaagugaugggccggcacaagcccgagaacaucgugaucgaaauggccagagagaaccagaccacccagaagggacagaagaacagccgcgagagaaugaagcggaucgaagagggcaucaaagagcugggcagccagauccugaaagaacaccccguggaaaacacccagcugcagaacgagaagcuguaccuguacuaccugcagaaugggcgggauauguacguggaccaggaacuggacaucaaccggcuguccgacuacgauguggaccauaucgugccucagagcuuucugaaggacgacuccaucgacaacaaggugcugaccagaagcgacaagaaccggggcaagagcgacaacgugcccuccgaagaggucgugaagaagaugaagaacuacuggcggcagcugcugaacgccaagcugauuacccagagaaaguucgacaaucugaccaaggccgagagaggcggccugagcgaacuggauaaggccggcuucaucaagagacagcugguggaaacccggcagaucacaaagcacguggcacagauccuggacucccggaugaacacuaaguacgacgagaaugacaagcugauccgggaagugaaagugaucacccugaaguccaagcugguguccgauuuccggaaggauuuccaguuuuacaaagugcgcgagaucaacaacuaccaccacgcccacgacgccuaccugaacgccgucgugggaaccgcccugaucaaaaaguacccuaagcuggaaagcgaguucguguacggcgacuacaagguguacgacgugcggaagaugaucgccaagagcgagcaggaaaucggcaaggcuaccgccaaguacuucuucuacagcaacaucaugaacuuuuucaagaccgagauuacccuggccaacggcgagauccggaagcggccucugaucgagacaaacggcgaaaccggggagaucgugugggauaagggccgggauuuugccaccgugcggaaagugcugagcaugccccaagugaauaucgugaaaaagaccgaggugcagacaggcggcuucagcaaagagucuauccugcccaagaggaacagcgauaagcugaucgccagaaagaaggacugggacccuaagaaguacggcggcuucgacagccccaccguggccuauucugugcuggugguggccaaaguggaaaagggcaaguccaagaaacugaagagugugaaagagcugcuggggaucaccaucauggaaagaagcagcuucgagaagaaucccaucgacuuucuggaagccaagggcuacaaagaagugaaaaaggaccugaucaucaagcugccuaaguacucccuguucgagcuggaaaacggccggaagagaaugcuggccucugccggcgaacugcagaagggaaacgaacuggcccugcccuccaaauaugugaacuuccuguaccuggccagccacuaugagaagcugaagggcucccccgaggauaaugagcagaaacagcuguuuguggaacagcacaagcacuaccuggacgagaucaucgagcagaucagcgaguucuccaagagagugauccuggccgacgcuaaucuggacaaagugcuguccgccuacaacaagcaccgggauaagcccaucagagagcaggccgagaauaucauccaccuguuuacccugaccaaucugggagccccugccgccuucaaguacuuugacaccaccaucgaccggaagagguacaccagcaccaaagaggugcuggacgccacccugauccaccagagcaucaccggccuguacgagacacggaucgaccugucucagcugggaggugacagcggcgggagcggcgggagcggggggagcacuaaucugagcgacaucauugagaaggagacugggaaacagcuggucauucaggaguccauccugaugcugccugaggagguggaggaagugaucggcaacaagccagagucugacauccuggugcacaccgccuacgacgaguccacagaugagaaugugaugcugcugaccucugacgcccccgaguauaagccuugggcccuggucauccaggauucuaacggcgagaauaagaucaagaugcugagcggaggauccggaggaucuggaggcagcaccaaccugucugacaucaucgagaaggagacaggcaagcagcuggucauccaggagagcauccugaugcugcccgaagaagucgaagaagugaucggaaacaagccugagagcgauauccugguccauaccgccuacgacgagaguaccgacgaaaaugugaugcugcugacauccgacgccccagaguauaagcccugggcucuggucauccaggauuccaacggagagaacaaaaucaaaaugcugucuggcggcucaaaaagaaccgccgacggcagcgaauucgagcccaagaagaagaggaaaguc

SEQ ID NO: 68 - DNA, 19 bp, Artificial Sequence
  Qbeta phage operator stem-loop seq
atgctgtctaagacagcat

SEQ ID NO: 69 - protein, 133 aa, Artificial Sequence
  Qbeta coat protein [Q65H] seq
MAKLETVTLGNIGKDGKQTLVLNPRGVNPTNGVASLSQAGAVPALEKRVTVSVSQPSRNRKNYKVHVKIQNPTACTANGSCDPSVTRQAYADVTFSFTQYSTDEERAFVRTELAALLASPLLIDAIDQLNPAY

SEQ ID NO: 70 - DNA, 15 bp, Artificial Sequence
  BoxB seq
gccctgaagaagggc

SEQ ID NO: 71 - protein, 22 aa, Artificial Sequence
  Lambda bacteriophage protein N (LambdaN-(1-22) seq
MNARTRRRERRAEKQAQWKAAN

SEQ ID NO: 72 - DNA, 16 bp, Artificial Sequence
  Csy4 binding motif
ctgccgtataggcagc

SEQ ID NO: 73 - protein, 187 aa, Artificial Sequence
  Csy4[H29A] seq
MDHYLDIRLRPDPEFPPAQLMSVLFGKLAQALVAQGGDRIGVSFPDLDESRSRLGERLRIHASADDLRALLARPWLEGLRDHLQFGEPAVVPHPTPYRQVSRVQAKSNPERLRRRLMRRHDLSEEEARKRIPDTVARALDLPFVTLRSQSTGQHFRLFIRHGPLQVTAEEGGFTCYGLSKGGFVPWF